European Patent Application EP 4 725 953 A1, published April 15, 2026. Title: Self-assembling peptides and hydrogels. Applicant: Max-Planck-Gesellschaft zur Förderung der Wissenschaften e.V. Application EP. The sequence listing filed with the application follows.

SEQUENCE LISTING (321 sequences)

SEQ ID NO: 1 - protein, 11 aa, synthetic construct
  VARIANT 3: note = K, R, or L
  VARIANT 11: note = M, M-NH2, or V
  VARIANT 1..3: note = may be deleted
  VARIANT 5: note = I or Y
  VARIANT 10..11: note = may be deleted
  VARIANT 11: note = may be deleted
GYXGXSLANWX

SEQ ID NO: 2 - protein, 6 aa, synthetic construct
GYLGIS

SEQ ID NO: 3 - protein, 6 aa, synthetic construct
GISLAN

SEQ ID NO: 4 - protein, 10 aa, synthetic construct
YRGISLANWM

SEQ ID NO: 5 - protein, 9 aa, synthetic construct
YRGISLANW

SEQ ID NO: 6 - protein, 11 aa, synthetic construct
GFRGISLANWM

SEQ ID NO: 7 - protein, 11 aa, synthetic construct
GYKGISLANWM

SEQ ID NO: 8 - protein, 11 aa, synthetic construct
GYRGISLANWM

SEQ ID NO: 9 - protein, 11 aa, synthetic construct
GYRGYSLANWM

SEQ ID NO: 10 - protein, 11 aa, synthetic construct
GYRGITLANWM

SEQ ID NO: 11 - protein, 11 aa, synthetic construct
GYRGISLAKWM

SEQ ID NO: 12 - protein, 11 aa, synthetic construct
GYRGISLANWV

SEQ ID NO: 13 - protein, 10 aa, synthetic construct
GYLGISLANW

SEQ ID NO: 14 - protein, 11 aa, synthetic construct
  SITE 11: note = Methionine Amide
GYRGISLANWM

SEQ ID NO: 15 - protein, 5 aa, synthetic construct
YRGIS

SEQ ID NO: 16 - protein, 6 aa, synthetic construct
SLANWM

SEQ ID NO: 17 - protein, 4 aa, synthetic construct
ISLA

SEQ ID NO: 18 - protein, 5 aa, synthetic construct
ISLAN

SEQ ID NO: 19 - protein, 5 aa, synthetic construct
GYRGI

SEQ ID NO: 20 - protein, 4 aa, synthetic construct
LANW

SEQ ID NO: 21 - protein, 5 aa, synthetic construct
RGISL

SEQ ID NO: 22 - protein, 11 aa, synthetic construct
GIRGISLANIM

SEQ ID NO: 23 - protein, 11 aa, synthetic construct
GKRGISLANWM

SEQ ID NO: 24 - protein, 11 aa, synthetic construct
GYVGISLANWM

SEQ ID NO: 25 - protein, 11 aa, synthetic construct
GYEGISLANWM

SEQ ID NO: 26 - protein, 11 aa, synthetic construct
GYRGISFANWM

SEQ ID NO: 27 - protein, 11 aa, synthetic construct
GYRGISLAEWM

SEQ ID NO: 28 - protein, 11 aa, synthetic construct
KYKGISLANWM

SEQ ID NO: 29 - protein, 11 aa, synthetic construct
GYRGISLFNWM

SEQ ID NO: 30 - protein, 6 aa, synthetic construct
GISLAL

SEQ ID NO: 31 - protein, 11 aa, synthetic construct
  VARIANT 1: note = G or A
  VARIANT 2: note = Y, F, or W
  VARIANT 3: note = R, K or L
  VARIANT 8: note = A, G, or V
  VARIANT 9: note = K, N, or Q
  VARIANT 10: note = W or F
  VARIANT 11: note = M, M-NH2, L, I, V, A, or G
  VARIANT 1..3: note = may be deleted
  VARIANT 1..2: note = may be deleted
  VARIANT 1: note = may be deleted
  VARIANT 8..11: note = may be deleted
  VARIANT 9..11: note = may be deleted
  VARIANT 10..11: note = may be deleted
  VARIANT 11: note = may be deleted
XXXGYSLXXXX

SEQ ID NO: 32 - protein, 11 aa, synthetic construct
  VARIANT 1: note = G or A
  VARIANT 2: note = Y, F, or W
  VARIANT 3: note = R, K or L
  VARIANT 8: note = A, G, or V
  VARIANT 9: note = K, N, or Q
  VARIANT 10: note = W or F
  VARIANT 11: note = M, M-NH2, L, I, V, A, or G
  VARIANT 1..3: note = may be deleted
  VARIANT 1..2: note = may be deleted
  VARIANT 1: note = may be deleted
  VARIANT 8..11: note = may be deleted
  VARIANT 9..11: note = may be deleted
  VARIANT 10..11: note = may be deleted
  VARIANT 11: note = may be deleted
XXXGISLXXXX

SEQ ID NO: 33 - protein, 11 aa, synthetic construct
  VARIANT 1: note = G or A
  VARIANT 2: note = Y, F, or W
  VARIANT 3: note = R, K or L
  VARIANT 8: note = A, G, or V
  VARIANT 9: note = K, N, or Q
  VARIANT 10: note = W or F
  VARIANT 11: note = M, M-NH2, L, I, V, A, or G
  VARIANT 1..3: note = may be deleted
  VARIANT 1..2: note = may be deleted
  VARIANT 1: note = may be deleted
  VARIANT 8..11: note = may be deleted
  VARIANT 9..11: note = may be deleted
  VARIANT 10..11: note = may be deleted
  VARIANT 11: note = may be deleted
XXXGYTLXXXX

SEQ ID NO: 34 - protein, 11 aa, synthetic construct
  VARIANT 1: note = G or A
  VARIANT 2: note = Y, F, or W
  VARIANT 3: note = R, K or L
  VARIANT 8: note = A, G, or V
  VARIANT 9: note = K, N, or Q
  VARIANT 10: note = W or F
  VARIANT 11: note = M, M-NH2, L, I, V, A, or G
  VARIANT 1..3: note = may be deleted
  VARIANT 1..2: note = may be deleted
  VARIANT 1: note = may be deleted
  VARIANT 8..11: note = may be deleted
  VARIANT 9..11: note = may be deleted
  VARIANT 10..11: note = may be deleted
  VARIANT 11: note = may be deleted
XXXGITLXXXX

SEQ ID NO: 35 - protein, 11 aa, synthetic construct
  VARIANT 1: note = G or A
  VARIANT 2: note = Y, F, or W
  VARIANT 3: note = R, K or L
  VARIANT 9: note = K, N, or Q
  VARIANT 10: note = W or F
  VARIANT 11: note = M, M-NH2, L, I, V, A, or G
  VARIANT 1..3: note = may be deleted
  VARIANT 1..2: note = may be deleted
  VARIANT 1: note = may be deleted
  VARIANT 9..11: note = may be deleted
  VARIANT 10..11: note = may be deleted
  VARIANT 11: note = may be deleted
  VARIANT 6: note = S or T
XXXGIXLAXXX

SEQ ID NO: 36 - protein, 11 aa, synthetic construct
  VARIANT 1: note = G or A
  VARIANT 2: note = Y, F, or W
  VARIANT 3: note = R, K or L
  VARIANT 9: note = K, N, or Q
  VARIANT 10: note = W or F
  VARIANT 11: note = M, M-NH2, L, I, V, A, or G
  VARIANT 1..3: note = may be deleted
  VARIANT 1..2: note = may be deleted
  VARIANT 1: note = may be deleted
  VARIANT 9..11: note = may be deleted
  VARIANT 10..11: note = may be deleted
  VARIANT 11: note = may be deleted
  VARIANT 6: note = S or T
XXXGYXLAXXX

SEQ ID NO: 37 - protein, 11 aa, synthetic construct
  VARIANT 1: note = G or A
  VARIANT 2: note = Y, F, or W
  VARIANT 3: note = R, K or L
  VARIANT 9: note = K, N, or Q
  VARIANT 10: note = W or F
  VARIANT 11: note = M, M-NH2, L, I, V, A, or G
  VARIANT 1..3: note = may be deleted
  VARIANT 1..2: note = may be deleted
  VARIANT 1: note = may be deleted
  VARIANT 9..11: note = may be deleted
  VARIANT 10..11: note = may be deleted
  VARIANT 11: note = may be deleted
  VARIANT 5: note = I, Y, Q, N, L, or F
XXXGXSLAXXX

SEQ ID NO: 38 - protein, 11 aa, synthetic construct
  VARIANT 1: note = G or A
  VARIANT 2: note = Y, F, or W
  VARIANT 3: note = R, K or L
  VARIANT 9: note = K, N, or Q
  VARIANT 10: note = W or F
  VARIANT 11: note = M, M-NH2, L, I, V, A, or G
  VARIANT 1..3: note = may be deleted
  VARIANT 1..2: note = may be deleted
  VARIANT 1: note = may be deleted
  VARIANT 9..11: note = may be deleted
  VARIANT 10..11: note = may be deleted
  VARIANT 11: note = may be deleted
  VARIANT 5: note = I, Y, Q, N, L, or F
XXXGXTLAXXX

SEQ ID NO: 39 - protein, 11 aa, synthetic construct
  VARIANT 1: note = G or A
  VARIANT 2: note = Y, F, or W
  VARIANT 3: note = R, K or L
  VARIANT 9: note = K, N, or Q
  VARIANT 10: note = W or F
  VARIANT 11: note = M, M-NH2, L, I, V, A, or G
  VARIANT 1..3: note = may be deleted
  VARIANT 1..2: note = may be deleted
  VARIANT 1: note = may be deleted
  VARIANT 9..11: note = may be deleted
  VARIANT 10..11: note = may be deleted
  VARIANT 11: note = may be deleted
  VARIANT 4: note = G or A
XXXXISLAXXX

SEQ ID NO: 40 - protein, 11 aa, synthetic construct
  VARIANT 1: note = G or A
  VARIANT 2: note = Y, F, or W
  VARIANT 3: note = R, K or L
  VARIANT 9: note = K, N, or Q
  VARIANT 10: note = W or F
  VARIANT 11: note = M, M-NH2, L, I, V, A, or G
  VARIANT 1..3: note = may be deleted
  VARIANT 1..2: note = may be deleted
  VARIANT 1: note = may be deleted
  VARIANT 9..11: note = may be deleted
  VARIANT 10..11: note = may be deleted
  VARIANT 11: note = may be deleted
  VARIANT 4: note = G or A
XXXXITLAXXX

SEQ ID NO: 41 - protein, 11 aa, synthetic construct
  VARIANT 1: note = G or A
  VARIANT 2: note = Y, F, or W
  VARIANT 3: note = R, K or L
  VARIANT 9: note = K, N, or Q
  VARIANT 10: note = W or F
  VARIANT 11: note = M, M-NH2, L, I, V, A, or G
  VARIANT 1..3: note = may be deleted
  VARIANT 1..2: note = may be deleted
  VARIANT 1: note = may be deleted
  VARIANT 9..11: note = may be deleted
  VARIANT 10..11: note = may be deleted
  VARIANT 11: note = may be deleted
  VARIANT 4: note = G or A
XXXXYSLAXXX

SEQ ID NO: 42 - protein, 11 aa, synthetic construct
  VARIANT 1: note = G or A
  VARIANT 2: note = Y, F, or W
  VARIANT 3: note = R, K or L
  VARIANT 9: note = K, N, or Q
  VARIANT 10: note = W or F
  VARIANT 11: note = M, M-NH2, L, I, V, A, or G
  VARIANT 1..3: note = may be deleted
  VARIANT 1..2: note = may be deleted
  VARIANT 1: note = may be deleted
  VARIANT 9..11: note = may be deleted
  VARIANT 10..11: note = may be deleted
  VARIANT 11: note = may be deleted
  VARIANT 4: note = G or A
XXXXYTLAXXX

SEQ ID NO: 43 - protein, 11 aa, synthetic construct
  VARIANT 1: note = G or A
  VARIANT 2: note = Y, F, or W
  VARIANT 3: note = R, K or L
  VARIANT 9: note = K, N, or Q
  VARIANT 10: note = W or F
  VARIANT 11: note = M, M-NH2, L, I, V, A, or G
  VARIANT 1..3: note = may be deleted
  VARIANT 1..2: note = may be deleted
  VARIANT 1: note = may be deleted
  VARIANT 9..11: note = may be deleted
  VARIANT 10..11: note = may be deleted
  VARIANT 11: note = may be deleted
XXXGYSLAXXX

SEQ ID NO: 44 - protein, 11 aa, synthetic construct
  VARIANT 1: note = G or A
  VARIANT 2: note = Y, F, or W
  VARIANT 3: note = R, K or L
  VARIANT 9: note = K, N, or Q
  VARIANT 10: note = W or F
  VARIANT 11: note = M, M-NH2, L, I, V, A, or G
  VARIANT 1..3: note = may be deleted
  VARIANT 1..2: note = may be deleted
  VARIANT 1: note = may be deleted
  VARIANT 9..11: note = may be deleted
  VARIANT 10..11: note = may be deleted
  VARIANT 11: note = may be deleted
  VARIANT 6: note = S or T
XXXGISLAXXX

SEQ ID NO: 45 - protein, 11 aa, synthetic construct
  VARIANT 1: note = G or A
  VARIANT 2: note = Y, F, or W
  VARIANT 3: note = R, K or L
  VARIANT 9: note = K, N, or Q
  VARIANT 10: note = W or F
  VARIANT 11: note = M, M-NH2, L, I, V, A, or G
  VARIANT 1..3: note = may be deleted
  VARIANT 1..2: note = may be deleted
  VARIANT 1: note = may be deleted
  VARIANT 9..11: note = may be deleted
  VARIANT 10..11: note = may be deleted
  VARIANT 11: note = may be deleted
XXXGYTLAXXX

SEQ ID NO: 46 - protein, 11 aa, synthetic construct
  VARIANT 1: note = G or A
  VARIANT 2: note = Y, F, or W
  VARIANT 3: note = R, K or L
  VARIANT 9: note = K, N, or Q
  VARIANT 10: note = W or F
  VARIANT 11: note = M, M-NH2, L, I, V, A, or G
  VARIANT 1..3: note = may be deleted
  VARIANT 1..2: note = may be deleted
  VARIANT 1: note = may be deleted
  VARIANT 9..11: note = may be deleted
  VARIANT 10..11: note = may be deleted
  VARIANT 11: note = may be deleted
XXXGITLAXXX

SEQ ID NO: 47 - protein, 11 aa, synthetic construct
  VARIANT 1: note = G or A
  VARIANT 2: note = Y, F, or W
  VARIANT 3: note = R, K or L
  VARIANT 10: note = W or F
  VARIANT 11: note = M, M-NH2, L, I, V, A, or G
  VARIANT 1..3: note = may be deleted
  VARIANT 1..2: note = may be deleted
  VARIANT 1: note = may be deleted
  VARIANT 10..11: note = may be deleted
  VARIANT 11: note = may be deleted
  VARIANT 6: note = S or T
XXXGIXLAKXX

SEQ ID NO: 48 - protein, 11 aa, synthetic construct
  VARIANT 1: note = G or A
  VARIANT 2: note = Y, F, or W
  VARIANT 3: note = R, K or L
  VARIANT 10: note = W or F
  VARIANT 11: note = M, M-NH2, L, I, V, A, or G
  VARIANT 1..3: note = may be deleted
  VARIANT 1..2: note = may be deleted
  VARIANT 1: note = may be deleted
  VARIANT 10..11: note = may be deleted
  VARIANT 11: note = may be deleted
  VARIANT 6: note = S or T
XXXGYXLAKXX

SEQ ID NO: 49 - protein, 11 aa, synthetic construct
  VARIANT 1: note = G or A
  VARIANT 2: note = Y, F, or W
  VARIANT 3: note = R, K or L
  VARIANT 10: note = W or F
  VARIANT 11: note = M, M-NH2, L, I, V, A, or G
  VARIANT 1..3: note = may be deleted
  VARIANT 1..2: note = may be deleted
  VARIANT 1: note = may be deleted
  VARIANT 10..11: note = may be deleted
  VARIANT 11: note = may be deleted
  VARIANT 5: note = I, Y, Q, N, L, or F
XXXGXSLAKXX

SEQ ID NO: 50 - protein, 11 aa, synthetic construct
  VARIANT 1: note = G or A
  VARIANT 2: note = Y, F, or W
  VARIANT 3: note = R, K or L
  VARIANT 10: note = W or F
  VARIANT 11: note = M, M-NH2, L, I, V, A, or G
  VARIANT 1..3: note = may be deleted
  VARIANT 1..2: note = may be deleted
  VARIANT 1: note = may be deleted
  VARIANT 10..11: note = may be deleted
  VARIANT 11: note = may be deleted
  VARIANT 5: note = I, Y, Q, N, L, or F
XXXGXTLAKXX

SEQ ID NO: 51 - protein, 11 aa, synthetic construct
  VARIANT 1: note = G or A
  VARIANT 2: note = Y, F, or W
  VARIANT 3: note = R, K or L
  VARIANT 10: note = W or F
  VARIANT 11: note = M, M-NH2, L, I, V, A, or G
  VARIANT 1..3: note = may be deleted
  VARIANT 1..2: note = may be deleted
  VARIANT 1: note = may be deleted
  VARIANT 10..11: note = may be deleted
  VARIANT 11: note = may be deleted
  VARIANT 4: note = G or A
XXXXISLAKXX

SEQ ID NO: 52 - protein, 11 aa, synthetic construct
  VARIANT 1: note = G or A
  VARIANT 2: note = Y, F, or W
  VARIANT 3: note = R, K or L
  VARIANT 10: note = W or F
  VARIANT 11: note = M, M-NH2, L, I, V, A, or G
  VARIANT 1..3: note = may be deleted
  VARIANT 1..2: note = may be deleted
  VARIANT 1: note = may be deleted
  VARIANT 10..11: note = may be deleted
  VARIANT 11: note = may be deleted
  VARIANT 4: note = G or A
XXXXITLAKXX

SEQ ID NO: 53 - protein, 11 aa, synthetic construct
  VARIANT 1: note = G or A
  VARIANT 2: note = Y, F, or W
  VARIANT 3: note = R, K or L
  VARIANT 10: note = W or F
  VARIANT 11: note = M, M-NH2, L, I, V, A, or G
  VARIANT 1..3: note = may be deleted
  VARIANT 1..2: note = may be deleted
  VARIANT 1: note = may be deleted
  VARIANT 10..11: note = may be deleted
  VARIANT 11: note = may be deleted
  VARIANT 4: note = G or A
XXXXYSLAKXX

SEQ ID NO: 54 - protein, 11 aa, synthetic construct
  VARIANT 1: note = G or A
  VARIANT 2: note = Y, F, or W
  VARIANT 3: note = R, K or L
  VARIANT 10: note = W or F
  VARIANT 11: note = M, M-NH2, L, I, V, A, or G
  VARIANT 1..3: note = may be deleted
  VARIANT 1..2: note = may be deleted
  VARIANT 1: note = may be deleted
  VARIANT 10..11: note = may be deleted
  VARIANT 11: note = may be deleted
  VARIANT 4: note = G or A
XXXXYTLAKXX

SEQ ID NO: 55 - protein, 11 aa, synthetic construct
  VARIANT 1: note = G or A
  VARIANT 2: note = Y, F, or W
  VARIANT 3: note = R, K or L
  VARIANT 10: note = W or F
  VARIANT 11: note = M, M-NH2, L, I, V, A, or G
  VARIANT 1..3: note = may be deleted
  VARIANT 1..2: note = may be deleted
  VARIANT 1: note = may be deleted
  VARIANT 10..11: note = may be deleted
  VARIANT 11: note = may be deleted
XXXGYSLAKXX

SEQ ID NO: 56 - protein, 11 aa, synthetic construct
  VARIANT 1: note = G or A
  VARIANT 2: note = Y, F, or W
  VARIANT 3: note = R, K or L
  VARIANT 10: note = W or F
  VARIANT 11: note = M, M-NH2, L, I, V, A, or G
  VARIANT 1..3: note = may be deleted
  VARIANT 1..2: note = may be deleted
  VARIANT 1: note = may be deleted
  VARIANT 10..11: note = may be deleted
  VARIANT 11: note = may be deleted
  VARIANT 6: note = S or T
XXXGISLAKXX

SEQ ID NO: 57 - protein, 11 aa, synthetic construct
  VARIANT 1: note = G or A
  VARIANT 2: note = Y, F, or W
  VARIANT 3: note = R, K or L
  VARIANT 10: note = W or F
  VARIANT 11: note = M, M-NH2, L, I, V, A, or G
  VARIANT 1..3: note = may be deleted
  VARIANT 1..2: note = may be deleted
  VARIANT 1: note = may be deleted
  VARIANT 10..11: note = may be deleted
  VARIANT 11: note = may be deleted
XXXGYTLAKXX

SEQ ID NO: 58 - protein, 11 aa, synthetic construct
  VARIANT 1: note = G or A
  VARIANT 2: note = Y, F, or W
  VARIANT 3: note = R, K or L
  VARIANT 10: note = W or F
  VARIANT 11: note = M, M-NH2, L, I, V, A, or G
  VARIANT 1..3: note = may be deleted
  VARIANT 1..2: note = may be deleted
  VARIANT 1: note = may be deleted
  VARIANT 10..11: note = may be deleted
  VARIANT 11: note = may be deleted
XXXGITLAKXX

SEQ ID NO: 59 - protein, 11 aa, synthetic construct
  VARIANT 1: note = G or A
  VARIANT 2: note = Y, F, or W
  VARIANT 3: note = R, K or L
  VARIANT 10: note = W or F
  VARIANT 11: note = M, M-NH2, L, I, V, A, or G
  VARIANT 1..3: note = may be deleted
  VARIANT 1..2: note = may be deleted
  VARIANT 1: note = may be deleted
  VARIANT 10..11: note = may be deleted
  VARIANT 11: note = may be deleted
  VARIANT 6: note = S or T
XXXGIXLANXX

SEQ ID NO: 60 - protein, 11 aa, synthetic construct
  VARIANT 1: note = G or A
  VARIANT 2: note = Y, F, or W
  VARIANT 3: note = R, K or L
  VARIANT 10: note = W or F
  VARIANT 11: note = M, M-NH2, L, I, V, A, or G
  VARIANT 1..3: note = may be deleted
  VARIANT 1..2: note = may be deleted
  VARIANT 1: note = may be deleted
  VARIANT 10..11: note = may be deleted
  VARIANT 11: note = may be deleted
  VARIANT 6: note = S or T
XXXGYXLANXX

SEQ ID NO: 61 - protein, 11 aa, synthetic construct
  VARIANT 1: note = G or A
  VARIANT 2: note = Y, F, or W
  VARIANT 3: note = R, K or L
  VARIANT 10: note = W or F
  VARIANT 11: note = M, M-NH2, L, I, V, A, or G
  VARIANT 1..3: note = may be deleted
  VARIANT 1..2: note = may be deleted
  VARIANT 1: note = may be deleted
  VARIANT 10..11: note = may be deleted
  VARIANT 11: note = may be deleted
  VARIANT 5: note = I, Y, Q, N, L, or F
XXXGXSLANXX

SEQ ID NO: 62 - protein, 11 aa, synthetic construct
  VARIANT 1: note = G or A
  VARIANT 2: note = Y, F, or W
  VARIANT 3: note = R, K or L
  VARIANT 10: note = W or F
  VARIANT 11: note = M, M-NH2, L, I, V, A, or G
  VARIANT 1..3: note = may be deleted
  VARIANT 1..2: note = may be deleted
  VARIANT 1: note = may be deleted
  VARIANT 10..11: note = may be deleted
  VARIANT 11: note = may be deleted
  VARIANT 5: note = I, Y, Q, N, L, or F
XXXGXTLANXX

SEQ ID NO: 63 - protein, 11 aa, synthetic construct
  VARIANT 1: note = G or A
  VARIANT 2: note = Y, F, or W
  VARIANT 3: note = R, K or L
  VARIANT 10: note = W or F
  VARIANT 11: note = M, M-NH2, L, I, V, A, or G
  VARIANT 1..3: note = may be deleted
  VARIANT 1..2: note = may be deleted
  VARIANT 1: note = may be deleted
  VARIANT 10..11: note = may be deleted
  VARIANT 11: note = may be deleted
  VARIANT 4: note = G or A
XXXXISLANXX

SEQ ID NO: 64 - protein, 11 aa, synthetic construct
  VARIANT 1: note = G or A
  VARIANT 2: note = Y, F, or W
  VARIANT 3: note = R, K or L
  VARIANT 10: note = W or F
  VARIANT 11: note = M, M-NH2, L, I, V, A, or G
  VARIANT 1..3: note = may be deleted
  VARIANT 1..2: note = may be deleted
  VARIANT 1: note = may be deleted
  VARIANT 10..11: note = may be deleted
  VARIANT 11: note = may be deleted
  VARIANT 4: note = G or A
XXXXITLANXX

SEQ ID NO: 65 - protein, 11 aa, synthetic construct
  VARIANT 1: note = G or A
  VARIANT 2: note = Y, F, or W
  VARIANT 3: note = R, K or L
  VARIANT 10: note = W or F
  VARIANT 11: note = M, M-NH2, L, I, V, A, or G
  VARIANT 1..3: note = may be deleted
  VARIANT 1..2: note = may be deleted
  VARIANT 1: note = may be deleted
  VARIANT 10..11: note = may be deleted
  VARIANT 11: note = may be deleted
  VARIANT 4: note = G or A
XXXXYSLANXX

SEQ ID NO: 66 - protein, 11 aa, synthetic construct
  VARIANT 1: note = G or A
  VARIANT 2: note = Y, F, or W
  VARIANT 3: note = R, K or L
  VARIANT 10: note = W or F
  VARIANT 11: note = M, M-NH2, L, I, V, A, or G
  VARIANT 1..3: note = may be deleted
  VARIANT 1..2: note = may be deleted
  VARIANT 1: note = may be deleted
  VARIANT 10..11: note = may be deleted
  VARIANT 11: note = may be deleted
  VARIANT 4: note = G or A
XXXXYTLANXX

SEQ ID NO: 67 - protein, 11 aa, synthetic construct
  VARIANT 1: note = G or A
  VARIANT 2: note = Y, F, or W
  VARIANT 3: note = R, K or L
  VARIANT 10: note = W or F
  VARIANT 11: note = M, M-NH2, L, I, V, A, or G
  VARIANT 1..3: note = may be deleted
  VARIANT 1..2: note = may be deleted
  VARIANT 1: note = may be deleted
  VARIANT 10..11: note = may be deleted
  VARIANT 11: note = may be deleted
XXXGYSLANXX

SEQ ID NO: 68 - protein, 11 aa, synthetic construct
  VARIANT 1: note = G or A
  VARIANT 2: note = Y, F, or W
  VARIANT 3: note = R, K or L
  VARIANT 10: note = W or F
  VARIANT 11: note = M, M-NH2, L, I, V, A, or G
  VARIANT 1..3: note = may be deleted
  VARIANT 1..2: note = may be deleted
  VARIANT 1: note = may be deleted
  VARIANT 10..11: note = may be deleted
  VARIANT 11: note = may be deleted
  VARIANT 6: note = S or T
XXXGISLANXX

SEQ ID NO: 69 - protein, 11 aa, synthetic construct
  VARIANT 1: note = G or A
  VARIANT 2: note = Y, F, or W
  VARIANT 3: note = R, K or L
  VARIANT 10: note = W or F
  VARIANT 11: note = M, M-NH2, L, I, V, A, or G
  VARIANT 1..3: note = may be deleted
  VARIANT 1..2: note = may be deleted
  VARIANT 1: note = may be deleted
  VARIANT 10..11: note = may be deleted
  VARIANT 11: note = may be deleted
XXXGYTLANXX

SEQ ID NO: 70 - protein, 11 aa, synthetic construct
  VARIANT 1: note = G or A
  VARIANT 2: note = Y, F, or W
  VARIANT 3: note = R, K or L
  VARIANT 10: note = W or F
  VARIANT 11: note = M, M-NH2, L, I, V, A, or G
  VARIANT 1..3: note = may be deleted
  VARIANT 1..2: note = may be deleted
  VARIANT 1: note = may be deleted
  VARIANT 10..11: note = may be deleted
  VARIANT 11: note = may be deleted
XXXGITLANXX

SEQ ID NO: 71 - protein, 11 aa, synthetic construct
  VARIANT 1: note = G or A
  VARIANT 2: note = Y, F, or W
  VARIANT 3: note = R, K or L
  VARIANT 11: note = M, M-NH2, L, I, V, A, or G
  VARIANT 1..3: note = may be deleted
  VARIANT 1..2: note = may be deleted
  VARIANT 1: note = may be deleted
  VARIANT 11: note = may be deleted
  VARIANT 6: note = S or T
XXXGIXLANWX

SEQ ID NO: 72 - protein, 11 aa, synthetic construct
  VARIANT 1: note = G or A
  VARIANT 2: note = Y, F, or W
  VARIANT 3: note = R, K or L
  VARIANT 11: note = M, M-NH2, L, I, V, A, or G
  VARIANT 1..3: note = may be deleted
  VARIANT 1..2: note = may be deleted
  VARIANT 1: note = may be deleted
  VARIANT 11: note = may be deleted
  VARIANT 6: note = S or T
XXXGYXLANWX

SEQ ID NO: 73 - protein, 11 aa, synthetic construct
  VARIANT 1: note = G or A
  VARIANT 2: note = Y, F, or W
  VARIANT 3: note = R, K or L
  VARIANT 11: note = M, M-NH2, L, I, V, A, or G
  VARIANT 1..3: note = may be deleted
  VARIANT 1..2: note = may be deleted
  VARIANT 1: note = may be deleted
  VARIANT 11: note = may be deleted
  VARIANT 5: note = I, Y, Q, N, L, or F
XXXGXSLANWX

SEQ ID NO: 74 - protein, 11 aa, synthetic construct
  VARIANT 1: note = G or A
  VARIANT 2: note = Y, F, or W
  VARIANT 3: note = R, K or L
  VARIANT 11: note = M, M-NH2, L, I, V, A, or G
  VARIANT 1..3: note = may be deleted
  VARIANT 1..2: note = may be deleted
  VARIANT 1: note = may be deleted
  VARIANT 11: note = may be deleted
  VARIANT 5: note = I, Y, Q, N, L, or F
XXXGXTLANWX

SEQ ID NO: 75 - protein, 11 aa, synthetic construct
  VARIANT 1: note = G or A
  VARIANT 2: note = Y, F, or W
  VARIANT 3: note = R, K or L
  VARIANT 11: note = M, M-NH2, L, I, V, A, or G
  VARIANT 1..3: note = may be deleted
  VARIANT 1..2: note = may be deleted
  VARIANT 1: note = may be deleted
  VARIANT 11: note = may be deleted
  VARIANT 4: note = G or A
XXXXISLANWX

SEQ ID NO: 76 - protein, 11 aa, synthetic construct
  VARIANT 1: note = G or A
  VARIANT 2: note = Y, F, or W
  VARIANT 3: note = R, K or L
  VARIANT 11: note = M, M-NH2, L, I, V, A, or G
  VARIANT 1..3: note = may be deleted
  VARIANT 1..2: note = may be deleted
  VARIANT 1: note = may be deleted
  VARIANT 11: note = may be deleted
  VARIANT 4: note = G or A
XXXXITLANWX

SEQ ID NO: 77 - protein, 11 aa, synthetic construct
  VARIANT 1: note = G or A
  VARIANT 2: note = Y, F, or W
  VARIANT 3: note = R, K or L
  VARIANT 11: note = M, M-NH2, L, I, V, A, or G
  VARIANT 1..3: note = may be deleted
  VARIANT 1..2: note = may be deleted
  VARIANT 1: note = may be deleted
  VARIANT 11: note = may be deleted
  VARIANT 4: note = G or A
XXXXYSLANWX

SEQ ID NO: 78 - protein, 11 aa, synthetic construct
  VARIANT 1: note = G or A
  VARIANT 2: note = Y, F, or W
  VARIANT 3: note = R, K or L
  VARIANT 11: note = M, M-NH2, L, I, V, A, or G
  VARIANT 1..3: note = may be deleted
  VARIANT 1..2: note = may be deleted
  VARIANT 1: note = may be deleted
  VARIANT 11: note = may be deleted
  VARIANT 4: note = G or A
XXXXYTLANWX

SEQ ID NO: 79 - protein, 11 aa, synthetic construct
  VARIANT 1: note = G or A
  VARIANT 2: note = Y, F, or W
  VARIANT 3: note = R, K or L
  VARIANT 11: note = M, M-NH2, L, I, V, A, or G
  VARIANT 1..3: note = may be deleted
  VARIANT 1..2: note = may be deleted
  VARIANT 1: note = may be deleted
  VARIANT 11: note = may be deleted
XXXGYSLANWX

SEQ ID NO: 80 - protein, 11 aa, synthetic construct
  VARIANT 1: note = G or A
  VARIANT 2: note = Y, F, or W
  VARIANT 3: note = R, K or L
  VARIANT 11: note = M, M-NH2, L, I, V, A, or G
  VARIANT 1..3: note = may be deleted
  VARIANT 1..2: note = may be deleted
  VARIANT 1: note = may be deleted
  VARIANT 11: note = may be deleted
  VARIANT 6: note = S or T
XXXGISLANWX

SEQ ID NO: 81 - protein, 11 aa, synthetic construct
  VARIANT 1: note = G or A
  VARIANT 2: note = Y, F, or W
  VARIANT 3: note = R, K or L
  VARIANT 11: note = M, M-NH2, L, I, V, A, or G
  VARIANT 1..3: note = may be deleted
  VARIANT 1..2: note = may be deleted
  VARIANT 1: note = may be deleted
  VARIANT 11: note = may be deleted
XXXGYTLANWX

SEQ ID NO: 82 - protein, 11 aa, synthetic construct
  VARIANT 1: note = G or A
  VARIANT 2: note = Y, F, or W
  VARIANT 3: note = R, K or L
  VARIANT 11: note = M, M-NH2, L, I, V, A, or G
  VARIANT 1..3: note = may be deleted
  VARIANT 1..2: note = may be deleted
  VARIANT 1: note = may be deleted
  VARIANT 11: note = may be deleted
XXXGITLANWX

SEQ ID NO: 83 - protein, 11 aa, synthetic construct
  VARIANT 1: note = G or A
  VARIANT 2: note = Y, F, or W
  VARIANT 3: note = R, K or L
  VARIANT 1..3: note = may be deleted
  VARIANT 1..2: note = may be deleted
  VARIANT 1: note = may be deleted
  VARIANT 6: note = S or T
XXXGIXLANWM

SEQ ID NO: 84 - protein, 11 aa, synthetic construct
  VARIANT 1: note = G or A
  VARIANT 2: note = Y, F, or W
  VARIANT 3: note = R, K or L
  VARIANT 1..3: note = may be deleted
  VARIANT 1..2: note = may be deleted
  VARIANT 1: note = may be deleted
  VARIANT 6: note = S or T
XXXGYXLANWM

SEQ ID NO: 85 - protein, 11 aa, synthetic construct
  VARIANT 1: note = G or A
  VARIANT 2: note = Y, F, or W
  VARIANT 3: note = R, K or L
  VARIANT 1..3: note = may be deleted
  VARIANT 1..2: note = may be deleted
  VARIANT 1: note = may be deleted
  VARIANT 5: note = I, Y, Q, N, L, or F
XXXGXSLANWM

SEQ ID NO: 86 - protein, 11 aa, synthetic construct
  VARIANT 1: note = G or A
  VARIANT 2: note = Y, F, or W
  VARIANT 3: note = R, K or L
  VARIANT 1..3: note = may be deleted
  VARIANT 1..2: note = may be deleted
  VARIANT 1: note = may be deleted
  VARIANT 5: note = I, Y, Q, N, L, or F
XXXGXTLANWM

SEQ ID NO: 87 - protein, 11 aa, synthetic construct
  VARIANT 1: note = G or A
  VARIANT 2: note = Y, F, or W
  VARIANT 3: note = R, K or L
  VARIANT 1..3: note = may be deleted
  VARIANT 1..2: note = may be deleted
  VARIANT 1: note = may be deleted
  VARIANT 4: note = G or A
XXXXISLANWM

SEQ ID NO: 88 - protein, 11 aa, synthetic construct
  VARIANT 1: note = G or A
  VARIANT 2: note = Y, F, or W
  VARIANT 3: note = R, K or L
  VARIANT 1..3: note = may be deleted
  VARIANT 1..2: note = may be deleted
  VARIANT 1: note = may be deleted
  VARIANT 4: note = G or A
XXXXITLANWM

SEQ ID NO: 89 - protein, 11 aa, synthetic construct
  VARIANT 1: note = G or A
  VARIANT 2: note = Y, F, or W
  VARIANT 3: note = R, K or L
  VARIANT 1..3: note = may be deleted
  VARIANT 1..2: note = may be deleted
  VARIANT 1: note = may be deleted
  VARIANT 4: note = G or A
XXXXYSLANWM

SEQ ID NO: 90 - protein, 11 aa, synthetic construct
  VARIANT 1: note = G or A
  VARIANT 2: note = Y, F, or W
  VARIANT 3: note = R, K or L
  VARIANT 1..3: note = may be deleted
  VARIANT 1..2: note = may be deleted
  VARIANT 1: note = may be deleted
  VARIANT 4: note = G or A
XXXXYTLANWM

SEQ ID NO: 91 - protein, 11 aa, synthetic construct
  VARIANT 1: note = G or A
  VARIANT 2: note = Y, F, or W
  VARIANT 3: note = R, K or L
  VARIANT 1..3: note = may be deleted
  VARIANT 1..2: note = may be deleted
  VARIANT 1: note = may be deleted
XXXGYSLANWM

SEQ ID NO: 92 - protein, 11 aa, synthetic construct
  VARIANT 1: note = G or A
  VARIANT 2: note = Y, F, or W
  VARIANT 3: note = R, K or L
  VARIANT 1..3: note = may be deleted
  VARIANT 1..2: note = may be deleted
  VARIANT 1: note = may be deleted
  VARIANT 6: note = S or T
XXXGISLANWM

SEQ ID NO: 93 - protein, 11 aa, synthetic construct
  VARIANT 1: note = G or A
  VARIANT 2: note = Y, F, or W
  VARIANT 3: note = R, K or L
  VARIANT 1..3: note = may be deleted
  VARIANT 1..2: note = may be deleted
  VARIANT 1: note = may be deleted
XXXGYTLANWM

SEQ ID NO: 94 - protein, 11 aa, synthetic construct
  VARIANT 1: note = G or A
  VARIANT 2: note = Y, F, or W
  VARIANT 3: note = R, K or L
  VARIANT 1..3: note = may be deleted
  VARIANT 1..2: note = may be deleted
  VARIANT 1: note = may be deleted
XXXGITLANWM

SEQ ID NO: 95 - protein, 11 aa, synthetic construct
  VARIANT 1: note = G or A
  VARIANT 2: note = Y, F, or W
  VARIANT 3: note = R, K or L
  VARIANT 1..3: note = may be deleted
  VARIANT 1..2: note = may be deleted
  VARIANT 1: note = may be deleted
  VARIANT 6: note = S or T
  SITE 11: note = Methionine Amide
XXXGIXLANWM

SEQ ID NO: 96 - protein, 11 aa, synthetic construct
  VARIANT 1: note = G or A
  VARIANT 2: note = Y, F, or W
  VARIANT 3: note = R, K or L
  VARIANT 1..3: note = may be deleted
  VARIANT 1..2: note = may be deleted
  VARIANT 1: note = may be deleted
  VARIANT 6: note = S or T
  SITE 11: note = Methionine Amide
XXXGYXLANWM

SEQ ID NO: 97 - protein, 11 aa, synthetic construct
  VARIANT 1: note = G or A
  VARIANT 2: note = Y, F, or W
  VARIANT 3: note = R, K or L
  VARIANT 1..3: note = may be deleted
  VARIANT 1..2: note = may be deleted
  VARIANT 1: note = may be deleted
  VARIANT 5: note = I, Y, Q, N, L, or F
  SITE 11: note = Methionine Amide
XXXGXSLANWM

SEQ ID NO: 98 - protein, 11 aa, synthetic construct
  VARIANT 1: note = G or A
  VARIANT 2: note = Y, F, or W
  VARIANT 3: note = R, K or L
  VARIANT 1..3: note = may be deleted
  VARIANT 1..2: note = may be deleted
  VARIANT 1: note = may be deleted
  VARIANT 5: note = I, Y, Q, N, L, or F
  SITE 11: note = Methionine Amide
XXXGXTLANWM

SEQ ID NO: 99 - protein, 11 aa, synthetic construct
  VARIANT 1: note = G or A
  VARIANT 2: note = Y, F, or W
  VARIANT 3: note = R, K or L
  VARIANT 1..3: note = may be deleted
  VARIANT 1..2: note = may be deleted
  VARIANT 1: note = may be deleted
  VARIANT 4: note = G or A
  SITE 11: note = Methionine Amide
XXXXISLANWM

SEQ ID NO: 100 - protein, 11 aa, synthetic construct
  VARIANT 1: note = G or A
  VARIANT 2: note = Y, F, or W
  VARIANT 3: note = R, K or L
  VARIANT 1..3: note = may be deleted
  VARIANT 1..2: note = may be deleted
  VARIANT 1: note = may be deleted
  VARIANT 4: note = G or A
  SITE 11: note = Methionine Amide
XXXXITLANWM

SEQ ID NO: 101 - protein, 11 aa, synthetic construct
  VARIANT 1: note = G or A
  VARIANT 2: note = Y, F, or W
  VARIANT 9: note = K, N, or Q
  VARIANT 10: note = W or F
  VARIANT 11: note = M, M-NH2, L, I, V, A, or G
  VARIANT 1..2: note = may be deleted
  VARIANT 1: note = may be deleted
  VARIANT 9..11: note = may be deleted
  VARIANT 10..11: note = may be deleted
  VARIANT 11: note = may be deleted
  VARIANT 5: note = I, Y, Q, N, L, or F
  VARIANT 8..11: note = may be deleted
  VARIANT 8: note = A, G or V
XXLGXSLXXXX

SEQ ID NO: 102 - protein, 11 aa, synthetic construct
  VARIANT 1: note = G or A
  VARIANT 2: note = Y, F, or W
  VARIANT 9: note = K, N, or Q
  VARIANT 10: note = W or F
  VARIANT 11: note = M, M-NH2, L, I, V, A, or G
  VARIANT 1..2: note = may be deleted
  VARIANT 1: note = may be deleted
  VARIANT 9..11: note = may be deleted
  VARIANT 10..11: note = may be deleted
  VARIANT 11: note = may be deleted
  VARIANT 5: note = I, Y, Q, N, L, or F
  VARIANT 8..11: note = may be deleted
  VARIANT 8: note = A, G or V
XXLGXTLXXXX

SEQ ID NO: 103 - protein, 11 aa, synthetic construct
  VARIANT 1: note = G or A
  VARIANT 2: note = Y, F, or W
  VARIANT 9: note = K, N, or Q
  VARIANT 10: note = W or F
  VARIANT 11: note = M, M-NH2, L, I, V, A, or G
  VARIANT 1..2: note = may be deleted
  VARIANT 1: note = may be deleted
  VARIANT 9..11: note = may be deleted
  VARIANT 10..11: note = may be deleted
  VARIANT 11: note = may be deleted
  VARIANT 8..11: note = may be deleted
  VARIANT 8: note = A, G or V
  VARIANT 4: note = G or A
XXLXISLXXXX

SEQ ID NO: 104 - protein, 11 aa, synthetic construct
  VARIANT 1: note = G or A
  VARIANT 2: note = Y, F, or W
  VARIANT 9: note = K, N, or Q
  VARIANT 10: note = W or F
  VARIANT 11: note = M, M-NH2, L, I, V, A, or G
  VARIANT 1..2: note = may be deleted
  VARIANT 1: note = may be deleted
  VARIANT 9..11: note = may be deleted
  VARIANT 10..11: note = may be deleted
  VARIANT 11: note = may be deleted
  VARIANT 8..11: note = may be deleted
  VARIANT 8: note = A, G or V
  VARIANT 4: note = G or A
XXLXITLXXXX

SEQ ID NO: 105 - protein, 11 aa, synthetic construct
  VARIANT 1: note = G or A
  VARIANT 2: note = Y, F, or W
  VARIANT 9: note = K, N, or Q
  VARIANT 10: note = W or F
  VARIANT 11: note = M, M-NH2, L, I, V, A, or G
  VARIANT 1..2: note = may be deleted
  VARIANT 1: note = may be deleted
  VARIANT 9..11: note = may be deleted
  VARIANT 10..11: note = may be deleted
  VARIANT 11: note = may be deleted
  VARIANT 8..11: note = may be deleted
  VARIANT 8: note = A, G or V
  VARIANT 4: note = G or A
XXLXYSLXXXX

SEQ ID NO: 106 - protein, 11 aa, synthetic construct
  VARIANT 1: note = G or A
  VARIANT 2: note = Y, F, or W
  VARIANT 9: note = K, N, or Q
  VARIANT 10: note = W or F
  VARIANT 11: note = M, M-NH2, L, I, V, A, or G
  VARIANT 1..2: note = may be deleted
  VARIANT 1: note = may be deleted
  VARIANT 9..11: note = may be deleted
  VARIANT 10..11: note = may be deleted
  VARIANT 11: note = may be deleted
  VARIANT 8..11: note = may be deleted
  VARIANT 8: note = A, G or V
  VARIANT 4: note = G or A
XXLXYTLXXXX

SEQ ID NO: 107 - protein, 11 aa, synthetic construct
  VARIANT 1: note = G or A
  VARIANT 2: note = Y, F, or W
  VARIANT 9: note = K, N, or Q
  VARIANT 10: note = W or F
  VARIANT 11: note = M, M-NH2, L, I, V, A, or G
  VARIANT 1..2: note = may be deleted
  VARIANT 1: note = may be deleted
  VARIANT 9..11: note = may be deleted
  VARIANT 10..11: note = may be deleted
  VARIANT 11: note = may be deleted
  VARIANT 8..11: note = may be deleted
  VARIANT 8: note = A, G or V
XXLGYSLXXXX

SEQ ID NO: 108 - protein, 11 aa, synthetic construct
  VARIANT 1: note = G or A
  VARIANT 2: note = Y, F, or W
  VARIANT 9: note = K, N, or Q
  VARIANT 10: note = W or F
  VARIANT 11: note = M, M-NH2, L, I, V, A, or G
  VARIANT 1..2: note = may be deleted
  VARIANT 1: note = may be deleted
  VARIANT 9..11: note = may be deleted
  VARIANT 10..11: note = may be deleted
  VARIANT 11: note = may be deleted
  VARIANT 8..11: note = may be deleted
  VARIANT 8: note = A, G or V
XXLGISLXXXX

SEQ ID NO: 109 - protein, 11 aa, synthetic construct
  VARIANT 1: note = G or A
  VARIANT 2: note = Y, F, or W
  VARIANT 9: note = K, N, or Q
  VARIANT 10: note = W or F
  VARIANT 11: note = M, M-NH2, L, I, V, A, or G
  VARIANT 1..2: note = may be deleted
  VARIANT 1: note = may be deleted
  VARIANT 9..11: note = may be deleted
  VARIANT 10..11: note = may be deleted
  VARIANT 11: note = may be deleted
  VARIANT 8..11: note = may be deleted
  VARIANT 8: note = A, G or V
XXLGYTLXXXX

SEQ ID NO: 110 - protein, 11 aa, synthetic construct
  VARIANT 1: note = G or A
  VARIANT 2: note = Y, F, or W
  VARIANT 9: note = K, N, or Q
  VARIANT 10: note = W or F
  VARIANT 11: note = M, M-NH2, L, I, V, A, or G
  VARIANT 1..2: note = may be deleted
  VARIANT 1: note = may be deleted
  VARIANT 9..11: note = may be deleted
  VARIANT 10..11: note = may be deleted
  VARIANT 11: note = may be deleted
  VARIANT 8..11: note = may be deleted
  VARIANT 8: note = A, G or V
XXLGITLXXXX

SEQ ID NO: 111 - protein, 11 aa, synthetic construct
  VARIANT 1: note = G or A
  VARIANT 2: note = Y, F, or W
  VARIANT 3: note = R, K or L
  VARIANT 1..3: note = may be deleted
  VARIANT 1..2: note = may be deleted
  VARIANT 1: note = may be deleted
  VARIANT 4: note = G or A
  SITE 11: note = Methionine Amide
XXXXYSLANWM

SEQ ID NO: 112 - protein, 11 aa, synthetic construct
  VARIANT 1: note = G or A
  VARIANT 2: note = Y, F, or W
  VARIANT 3: note = R, K or L
  VARIANT 1..3: note = may be deleted
  VARIANT 1..2: note = may be deleted
  VARIANT 1: note = may be deleted
  VARIANT 4: note = G or A
  SITE 11: note = Methionine Amide
XXXXYTLANWM

SEQ ID NO: 113 - protein, 11 aa, synthetic construct
  VARIANT 1: note = G or A
  VARIANT 2: note = Y, F, or W
  VARIANT 3: note = R, K or L
  VARIANT 1..3: note = may be deleted
  VARIANT 1..2: note = may be deleted
  VARIANT 1: note = may be deleted
  VARIANT 4: note = G or A
  SITE 11: note = Methionine Amide
XXXGYSLANWM

SEQ ID NO: 114 - protein, 11 aa, synthetic construct
  VARIANT 1: note = G or A
  VARIANT 2: note = Y, F, or W
  VARIANT 3: note = R, K or L
  VARIANT 1..3: note = may be deleted
  VARIANT 1..2: note = may be deleted
  VARIANT 1: note = may be deleted
  VARIANT 4: note = G or A
  SITE 11: note = Methionine Amide
XXXGISLANWM

SEQ ID NO: 115 - protein, 11 aa, synthetic construct
  VARIANT 1: note = G or A
  VARIANT 2: note = Y, F, or W
  VARIANT 3: note = R, K or L
  VARIANT 1..3: note = may be deleted
  VARIANT 1..2: note = may be deleted
  VARIANT 1: note = may be deleted
  VARIANT 4: note = G or A
  SITE 11: note = Methionine Amide
XXXGYTLANWM

SEQ ID NO: 116 - protein, 11 aa, synthetic construct
  VARIANT 1: note = G or A
  VARIANT 2: note = Y, F, or W
  VARIANT 3: note = R, K or L
  VARIANT 1..3: note = may be deleted
  VARIANT 1..2: note = may be deleted
  VARIANT 1: note = may be deleted
  VARIANT 4: note = G or A
  SITE 11: note = Methionine Amide
XXXGITLANWM

SEQ ID NO: 117 - protein, 11 aa, synthetic construct
  VARIANT 1: note = G or A
  VARIANT 2: note = Y, F, or W
  VARIANT 3: note = R, K or L
  VARIANT 1..3: note = may be deleted
  VARIANT 1..2: note = may be deleted
  VARIANT 1: note = may be deleted
  VARIANT 6: note = S or T
XXXGIXLANWV

SEQ ID NO: 118 - protein, 11 aa, synthetic construct
  VARIANT 1: note = G or A
  VARIANT 2: note = Y, F, or W
  VARIANT 3: note = R, K or L
  VARIANT 1..3: note = may be deleted
  VARIANT 1..2: note = may be deleted
  VARIANT 1: note = may be deleted
  VARIANT 6: note = S or T
XXXGYXLANWV

SEQ ID NO: 119 - protein, 11 aa, synthetic construct
  VARIANT 1: note = G or A
  VARIANT 2: note = Y, F, or W
  VARIANT 3: note = R, K or L
  VARIANT 1..3: note = may be deleted
  VARIANT 1..2: note = may be deleted
  VARIANT 1: note = may be deleted
  VARIANT 5: note = I, Y, Q, N, L, or F
XXXGXSLANWV

SEQ ID NO: 120 - protein, 11 aa, synthetic construct
  VARIANT 1: note = G or A
  VARIANT 2: note = Y, F, or W
  VARIANT 3: note = R, K or L
  VARIANT 1..3: note = may be deleted
  VARIANT 1..2: note = may be deleted
  VARIANT 1: note = may be deleted
  VARIANT 5: note = I, Y, Q, N, L, or F
XXXGXTLANWV

SEQ ID NO: 121 - protein, 11 aa, synthetic construct
  VARIANT 1: note = G or A
  VARIANT 2: note = Y, F, or W
  VARIANT 3: note = R, K or L
  VARIANT 1..3: note = may be deleted
  VARIANT 1..2: note = may be deleted
  VARIANT 1: note = may be deleted
  VARIANT 4: note = G or A
XXXXISLANWV

SEQ ID NO: 122 - protein, 11 aa, synthetic construct
  VARIANT 1: note = G or A
  VARIANT 2: note = Y, F, or W
  VARIANT 3: note = R, K or L
  VARIANT 1..3: note = may be deleted
  VARIANT 1..2: note = may be deleted
  VARIANT 1: note = may be deleted
  VARIANT 4: note = G or A
XXXXITLANWV

SEQ ID NO: 123 - protein, 11 aa, synthetic construct
  VARIANT 1: note = G or A
  VARIANT 2: note = Y, F, or W
  VARIANT 3: note = R, K or L
  VARIANT 1..3: note = may be deleted
  VARIANT 1..2: note = may be deleted
  VARIANT 1: note = may be deleted
  VARIANT 4: note = G or A
XXXXYSLANWV

SEQ ID NO: 124 - protein, 11 aa, synthetic construct
  VARIANT 1: note = G or A
  VARIANT 2: note = Y, F, or W
  VARIANT 3: note = R, K or L
  VARIANT 1..3: note = may be deleted
  VARIANT 1..2: note = may be deleted
  VARIANT 1: note = may be deleted
  VARIANT 4: note = G or A
XXXXYTLANWV

SEQ ID NO: 125 - protein, 11 aa, synthetic construct
  VARIANT 1: note = G or A
  VARIANT 2: note = Y, F, or W
  VARIANT 3: note = R, K or L
  VARIANT 1..3: note = may be deleted
  VARIANT 1..2: note = may be deleted
  VARIANT 1: note = may be deleted
XXXGYSLANWV

SEQ ID NO: 126 - protein, 11 aa, synthetic construct
  VARIANT 1: note = G or A
  VARIANT 2: note = Y, F, or W
  VARIANT 3: note = R, K or L
  VARIANT 1..3: note = may be deleted
  VARIANT 1..2: note = may be deleted
  VARIANT 1: note = may be deleted
  VARIANT 6: note = S or T
XXXGISLANWV

SEQ ID NO: 127 - protein, 11 aa, synthetic construct
  VARIANT 1: note = G or A
  VARIANT 2: note = Y, F, or W
  VARIANT 3: note = R, K or L
  VARIANT 1..3: note = may be deleted
  VARIANT 1..2: note = may be deleted
  VARIANT 1: note = may be deleted
XXXGYTLANWV

SEQ ID NO: 128 - protein, 11 aa, synthetic construct
  VARIANT 1: note = G or A
  VARIANT 2: note = Y, F, or W
  VARIANT 3: note = R, K or L
  VARIANT 1..3: note = may be deleted
  VARIANT 1..2: note = may be deleted
  VARIANT 1: note = may be deleted
XXXGITLANWV

SEQ ID NO: 129 - protein, 11 aa, synthetic construct
  VARIANT 1: note = G or A
  VARIANT 2: note = Y, F, or W
  VARIANT 8: note = A, G, or V
  VARIANT 9: note = K, N, or Q
  VARIANT 10: note = W or F
  VARIANT 11: note = M, M-NH2, L, I, V, A, or G
  VARIANT 1..2: note = may be deleted
  VARIANT 1: note = may be deleted
  VARIANT 8..11: note = may be deleted
  VARIANT 9..11: note = may be deleted
  VARIANT 10..11: note = may be deleted
  VARIANT 11: note = may be deleted
  VARIANT 7..11: note = may be deleted
  VARIANT 7: note = L, I, or V
XXRGYSXXXXX

SEQ ID NO: 130 - protein, 11 aa, synthetic construct
  VARIANT 1: note = G or A
  VARIANT 2: note = Y, F, or W
  VARIANT 8: note = A, G, or V
  VARIANT 9: note = K, N, or Q
  VARIANT 10: note = W or F
  VARIANT 11: note = M, M-NH2, L, I, V, A, or G
  VARIANT 1..2: note = may be deleted
  VARIANT 1: note = may be deleted
  VARIANT 8..11: note = may be deleted
  VARIANT 9..11: note = may be deleted
  VARIANT 10..11: note = may be deleted
  VARIANT 11: note = may be deleted
  VARIANT 7..11: note = may be deleted
  VARIANT 7: note = L, I, or V
XXRGISXXXXX

SEQ ID NO: 131 - protein, 11 aa, synthetic construct
  VARIANT 1: note = G or A
  VARIANT 2: note = Y, F, or W
  VARIANT 8: note = A, G, or V
  VARIANT 9: note = K, N, or Q
  VARIANT 10: note = W or F
  VARIANT 11: note = M, M-NH2, L, I, V, A, or G
  VARIANT 1..2: note = may be deleted
  VARIANT 1: note = may be deleted
  VARIANT 8..11: note = may be deleted
  VARIANT 9..11: note = may be deleted
  VARIANT 10..11: note = may be deleted
  VARIANT 11: note = may be deleted
  VARIANT 7..11: note = may be deleted
  VARIANT 7: note = L, I, or V
XXRGYTXXXXX

SEQ ID NO: 132 - protein, 11 aa, synthetic construct
  VARIANT 1: note = G or A
  VARIANT 2: note = Y, F, or W
  VARIANT 8: note = A, G, or V
  VARIANT 9: note = K, N, or Q
  VARIANT 10: note = W or F
  VARIANT 11: note = M, M-NH2, L, I, V, A, or G
  VARIANT 1..2: note = may be deleted
  VARIANT 1: note = may be deleted
  VARIANT 8..11: note = may be deleted
  VARIANT 9..11: note = may be deleted
  VARIANT 10..11: note = may be deleted
  VARIANT 11: note = may be deleted
  VARIANT 7..11: note = may be deleted
  VARIANT 7: note = L, I, or V
XXRGITXXXXX

SEQ ID NO: 133 - protein, 11 aa, synthetic construct
  VARIANT 1: note = G or A
  VARIANT 2: note = Y, F, or W
  VARIANT 8: note = A, G, or V
  VARIANT 9: note = K, N, or Q
  VARIANT 10: note = W or F
  VARIANT 11: note = M, M-NH2, L, I, V, A, or G
  VARIANT 1..2: note = may be deleted
  VARIANT 1: note = may be deleted
  VARIANT 8..11: note = may be deleted
  VARIANT 9..11: note = may be deleted
  VARIANT 10..11: note = may be deleted
  VARIANT 11: note = may be deleted
  VARIANT 7..11: note = may be deleted
  VARIANT 7: note = L, I, or V
XXKGYSXXXXX

SEQ ID NO: 134 - protein, 11 aa, synthetic construct
  VARIANT 1: note = G or A
  VARIANT 2: note = Y, F, or W
  VARIANT 8: note = A, G, or V
  VARIANT 9: note = K, N, or Q
  VARIANT 10: note = W or F
  VARIANT 11: note = M, M-NH2, L, I, V, A, or G
  VARIANT 1..2: note = may be deleted
  VARIANT 1: note = may be deleted
  VARIANT 8..11: note = may be deleted
  VARIANT 9..11: note = may be deleted
  VARIANT 10..11: note = may be deleted
  VARIANT 11: note = may be deleted
  VARIANT 7..11: note = may be deleted
  VARIANT 7: note = L, I, or V
XXKGISXXXXX

SEQ ID NO: 135 - protein, 11 aa, synthetic construct
  VARIANT 1: note = G or A
  VARIANT 2: note = Y, F, or W
  VARIANT 8: note = A, G, or V
  VARIANT 9: note = K, N, or Q
  VARIANT 10: note = W or F
  VARIANT 11: note = M, M-NH2, L, I, V, A, or G
  VARIANT 1..2: note = may be deleted
  VARIANT 1: note = may be deleted
  VARIANT 8..11: note = may be deleted
  VARIANT 9..11: note = may be deleted
  VARIANT 10..11: note = may be deleted
  VARIANT 11: note = may be deleted
  VARIANT 7..11: note = may be deleted
  VARIANT 7: note = L, I, or V
XXKGYTXXXXX

SEQ ID NO: 136 - protein, 11 aa, synthetic construct
  VARIANT 1: note = G or A
  VARIANT 2: note = Y, F, or W
  VARIANT 8: note = A, G, or V
  VARIANT 9: note = K, N, or Q
  VARIANT 10: note = W or F
  VARIANT 11: note = M, M-NH2, L, I, V, A, or G
  VARIANT 1..2: note = may be deleted
  VARIANT 1: note = may be deleted
  VARIANT 8..11: note = may be deleted
  VARIANT 9..11: note = may be deleted
  VARIANT 10..11: note = may be deleted
  VARIANT 11: note = may be deleted
  VARIANT 7..11: note = may be deleted
  VARIANT 7: note = L, I, or V
XXKGITXXXXX

SEQ ID NO: 137 - protein, 11 aa, synthetic construct
  VARIANT 1: note = G or A
  VARIANT 2: note = Y, F, or W
  VARIANT 8: note = A, G, or V
  VARIANT 9: note = K, N, or Q
  VARIANT 10: note = W or F
  VARIANT 11: note = M, M-NH2, L, I, V, A, or G
  VARIANT 1..2: note = may be deleted
  VARIANT 1: note = may be deleted
  VARIANT 8..11: note = may be deleted
  VARIANT 9..11: note = may be deleted
  VARIANT 10..11: note = may be deleted
  VARIANT 11: note = may be deleted
  VARIANT 7..11: note = may be deleted
  VARIANT 7: note = L, I, or V
XXLGYSXXXXX

SEQ ID NO: 138 - protein, 11 aa, synthetic construct
  VARIANT 1: note = G or A
  VARIANT 2: note = Y, F, or W
  VARIANT 8: note = A, G, or V
  VARIANT 9: note = K, N, or Q
  VARIANT 10: note = W or F
  VARIANT 11: note = M, M-NH2, L, I, V, A, or G
  VARIANT 1..2: note = may be deleted
  VARIANT 1: note = may be deleted
  VARIANT 8..11: note = may be deleted
  VARIANT 9..11: note = may be deleted
  VARIANT 10..11: note = may be deleted
  VARIANT 11: note = may be deleted
  VARIANT 7..11: note = may be deleted
  VARIANT 7: note = L, I, or V
XXLGISXXXXX

SEQ ID NO: 139 - protein, 11 aa, synthetic construct
  VARIANT 1: note = G or A
  VARIANT 2: note = Y, F, or W
  VARIANT 8: note = A, G, or V
  VARIANT 9: note = K, N, or Q
  VARIANT 10: note = W or F
  VARIANT 11: note = M, M-NH2, L, I, V, A, or G
  VARIANT 1..2: note = may be deleted
  VARIANT 1: note = may be deleted
  VARIANT 8..11: note = may be deleted
  VARIANT 9..11: note = may be deleted
  VARIANT 10..11: note = may be deleted
  VARIANT 11: note = may be deleted
  VARIANT 7..11: note = may be deleted
  VARIANT 7: note = L, I, or V
XXLGYTXXXXX

SEQ ID NO: 140 - protein, 11 aa, synthetic construct
  VARIANT 1: note = G or A
  VARIANT 2: note = Y, F, or W
  VARIANT 8: note = A, G, or V
  VARIANT 9: note = K, N, or Q
  VARIANT 10: note = W or F
  VARIANT 11: note = M, M-NH2, L, I, V, A, or G
  VARIANT 1..2: note = may be deleted
  VARIANT 1: note = may be deleted
  VARIANT 8..11: note = may be deleted
  VARIANT 9..11: note = may be deleted
  VARIANT 10..11: note = may be deleted
  VARIANT 11: note = may be deleted
  VARIANT 7..11: note = may be deleted
  VARIANT 7: note = L, I, or V
XXLGITXXXXX

SEQ ID NO: 141 - protein, 11 aa, synthetic construct
  VARIANT 1: note = G or A
  VARIANT 8: note = A, G, or V
  VARIANT 9: note = K, N, or Q
  VARIANT 10: note = W or F
  VARIANT 11: note = M, M-NH2, L, I, V, A, or G
  VARIANT 1: note = may be deleted
  VARIANT 8..11: note = may be deleted
  VARIANT 9..11: note = may be deleted
  VARIANT 10..11: note = may be deleted
  VARIANT 11: note = may be deleted
  VARIANT 7..11: note = may be deleted
  VARIANT 7: note = L, I, or V
  VARIANT 6: note = S or T
XYRGIXXXXXX

SEQ ID NO: 142 - protein, 11 aa, synthetic construct
  VARIANT 1: note = G or A
  VARIANT 8: note = A, G, or V
  VARIANT 9: note = K, N, or Q
  VARIANT 10: note = W or F
  VARIANT 11: note = M, M-NH2, L, I, V, A, or G
  VARIANT 1: note = may be deleted
  VARIANT 8..11: note = may be deleted
  VARIANT 9..11: note = may be deleted
  VARIANT 10..11: note = may be deleted
  VARIANT 11: note = may be deleted
  VARIANT 7..11: note = may be deleted
  VARIANT 7: note = L, I, or V
  VARIANT 6: note = S or T
XYRGYXXXXXX

SEQ ID NO: 143 - protein, 11 aa, synthetic construct
  VARIANT 1: note = G or A
  VARIANT 8: note = A, G, or V
  VARIANT 9: note = K, N, or Q
  VARIANT 10: note = W or F
  VARIANT 11: note = M, M-NH2, L, I, V, A, or G
  VARIANT 1: note = may be deleted
  VARIANT 8..11: note = may be deleted
  VARIANT 9..11: note = may be deleted
  VARIANT 10..11: note = may be deleted
  VARIANT 11: note = may be deleted
  VARIANT 7..11: note = may be deleted
  VARIANT 7: note = L, I, or V
  VARIANT 5: note = I, Y, Q, N, L, or F
XYRGXSXXXXX

SEQ ID NO: 144 - protein, 11 aa, synthetic construct
  VARIANT 1: note = G or A
  VARIANT 8: note = A, G, or V
  VARIANT 9: note = K, N, or Q
  VARIANT 10: note = W or F
  VARIANT 11: note = M, M-NH2, L, I, V, A, or G
  VARIANT 1: note = may be deleted
  VARIANT 8..11: note = may be deleted
  VARIANT 9..11: note = may be deleted
  VARIANT 10..11: note = may be deleted
  VARIANT 11: note = may be deleted
  VARIANT 7..11: note = may be deleted
  VARIANT 7: note = L, I, or V
  VARIANT 5: note = I, Y, Q, N, L, or F
XYRGXTXXXXX

SEQ ID NO: 145 - protein, 11 aa, synthetic construct
  VARIANT 1: note = G or A
  VARIANT 8: note = A, G, or V
  VARIANT 9: note = K, N, or Q
  VARIANT 10: note = W or F
  VARIANT 11: note = M, M-NH2, L, I, V, A, or G
  VARIANT 1: note = may be deleted
  VARIANT 8..11: note = may be deleted
  VARIANT 9..11: note = may be deleted
  VARIANT 10..11: note = may be deleted
  VARIANT 11: note = may be deleted
  VARIANT 7..11: note = may be deleted
  VARIANT 7: note = L, I, or V
  VARIANT 4: note = G or A
XYRXISXXXXX

SEQ ID NO: 146 - protein, 11 aa, synthetic construct
  VARIANT 1: note = G or A
  VARIANT 8: note = A, G, or V
  VARIANT 9: note = K, N, or Q
  VARIANT 10: note = W or F
  VARIANT 11: note = M, M-NH2, L, I, V, A, or G
  VARIANT 1: note = may be deleted
  VARIANT 8..11: note = may be deleted
  VARIANT 9..11: note = may be deleted
  VARIANT 10..11: note = may be deleted
  VARIANT 11: note = may be deleted
  VARIANT 7..11: note = may be deleted
  VARIANT 7: note = L, I, or V
  VARIANT 4: note = G or A
XYRXITXXXXX

SEQ ID NO: 147 - protein, 11 aa, synthetic construct
  VARIANT 1: note = G or A
  VARIANT 8: note = A, G, or V
  VARIANT 9: note = K, N, or Q
  VARIANT 10: note = W or F
  VARIANT 11: note = M, M-NH2, L, I, V, A, or G
  VARIANT 1: note = may be deleted
  VARIANT 8..11: note = may be deleted
  VARIANT 9..11: note = may be deleted
  VARIANT 10..11: note = may be deleted
  VARIANT 11: note = may be deleted
  VARIANT 7..11: note = may be deleted
  VARIANT 7: note = L, I, or V
  VARIANT 4: note = G or A
XYRXYSXXXXX

SEQ ID NO: 148 - protein, 11 aa, synthetic construct
  VARIANT 1: note = G or A
  VARIANT 8: note = A, G, or V
  VARIANT 9: note = K, N, or Q
  VARIANT 10: note = W or F
  VARIANT 11: note = M, M-NH2, L, I, V, A, or G
  VARIANT 1: note = may be deleted
  VARIANT 8..11: note = may be deleted
  VARIANT 9..11: note = may be deleted
  VARIANT 10..11: note = may be deleted
  VARIANT 11: note = may be deleted
  VARIANT 7..11: note = may be deleted
  VARIANT 7: note = L, I, or V
  VARIANT 4: note = G or A
XYRXYTXXXXX

SEQ ID NO: 149 - protein, 11 aa, synthetic construct
  VARIANT 1: note = G or A
  VARIANT 8: note = A, G, or V
  VARIANT 9: note = K, N, or Q
  VARIANT 10: note = W or F
  VARIANT 11: note = M, M-NH2, L, I, V, A, or G
  VARIANT 1: note = may be deleted
  VARIANT 8..11: note = may be deleted
  VARIANT 9..11: note = may be deleted
  VARIANT 10..11: note = may be deleted
  VARIANT 11: note = may be deleted
  VARIANT 7..11: note = may be deleted
  VARIANT 7: note = L, I, or V
XYRGYSXXXXX

SEQ ID NO: 150 - protein, 11 aa, synthetic construct
  VARIANT 1: note = G or A
  VARIANT 8: note = A, G, or V
  VARIANT 9: note = K, N, or Q
  VARIANT 10: note = W or F
  VARIANT 11: note = M, M-NH2, L, I, V, A, or G
  VARIANT 1: note = may be deleted
  VARIANT 8..11: note = may be deleted
  VARIANT 9..11: note = may be deleted
  VARIANT 10..11: note = may be deleted
  VARIANT 11: note = may be deleted
  VARIANT 7..11: note = may be deleted
  VARIANT 7: note = L, I, or V
XYRGISXXXXX

SEQ ID NO: 151 - protein, 11 aa, synthetic construct
  VARIANT 1: note = G or A
  VARIANT 8: note = A, G, or V
  VARIANT 9: note = K, N, or Q
  VARIANT 10: note = W or F
  VARIANT 11: note = M, M-NH2, L, I, V, A, or G
  VARIANT 1: note = may be deleted
  VARIANT 8..11: note = may be deleted
  VARIANT 9..11: note = may be deleted
  VARIANT 10..11: note = may be deleted
  VARIANT 11: note = may be deleted
  VARIANT 7..11: note = may be deleted
  VARIANT 7: note = L, I, or V
XYRGYTXXXXX

SEQ ID NO: 152 - protein, 11 aa, synthetic construct
  VARIANT 1: note = G or A
  VARIANT 8: note = A, G, or V
  VARIANT 9: note = K, N, or Q
  VARIANT 10: note = W or F
  VARIANT 11: note = M, M-NH2, L, I, V, A, or G
  VARIANT 1: note = may be deleted
  VARIANT 8..11: note = may be deleted
  VARIANT 9..11: note = may be deleted
  VARIANT 10..11: note = may be deleted
  VARIANT 11: note = may be deleted
  VARIANT 7..11: note = may be deleted
  VARIANT 7: note = L, I, or V
XYRGITXXXXX

SEQ ID NO: 153 - protein, 11 aa, synthetic construct
  VARIANT 1: note = G or A
  VARIANT 8: note = A, G, or V
  VARIANT 9: note = K, N, or Q
  VARIANT 10: note = W or F
  VARIANT 11: note = M, M-NH2, L, I, V, A, or G
  VARIANT 1: note = may be deleted
  VARIANT 8..11: note = may be deleted
  VARIANT 9..11: note = may be deleted
  VARIANT 10..11: note = may be deleted
  VARIANT 11: note = may be deleted
  VARIANT 7..11: note = may be deleted
  VARIANT 7: note = L, I, or V
  VARIANT 6: note = S or T
XYKGIXXXXXX

SEQ ID NO: 154 - protein, 11 aa, synthetic construct
  VARIANT 1: note = G or A
  VARIANT 8: note = A, G, or V
  VARIANT 9: note = K, N, or Q
  VARIANT 10: note = W or F
  VARIANT 11: note = M, M-NH2, L, I, V, A, or G
  VARIANT 1: note = may be deleted
  VARIANT 8..11: note = may be deleted
  VARIANT 9..11: note = may be deleted
  VARIANT 10..11: note = may be deleted
  VARIANT 11: note = may be deleted
  VARIANT 7..11: note = may be deleted
  VARIANT 7: note = L, I, or V
  VARIANT 6: note = S or T
XYKGYXXXXXX

SEQ ID NO: 155 - protein, 11 aa, synthetic construct
  VARIANT 1: note = G or A
  VARIANT 8: note = A, G, or V
  VARIANT 9: note = K, N, or Q
  VARIANT 10: note = W or F
  VARIANT 11: note = M, M-NH2, L, I, V, A, or G
  VARIANT 1: note = may be deleted
  VARIANT 8..11: note = may be deleted
  VARIANT 9..11: note = may be deleted
  VARIANT 10..11: note = may be deleted
  VARIANT 11: note = may be deleted
  VARIANT 7..11: note = may be deleted
  VARIANT 7: note = L, I, or V
  VARIANT 5: note = I, Y, Q, N, L, or F
XYKGXSXXXXX

SEQ ID NO: 156 - protein, 11 aa, synthetic construct
  VARIANT 1: note = G or A
  VARIANT 8: note = A, G, or V
  VARIANT 9: note = K, N, or Q
  VARIANT 10: note = W or F
  VARIANT 11: note = M, M-NH2, L, I, V, A, or G
  VARIANT 1: note = may be deleted
  VARIANT 8..11: note = may be deleted
  VARIANT 9..11: note = may be deleted
  VARIANT 10..11: note = may be deleted
  VARIANT 11: note = may be deleted
  VARIANT 7..11: note = may be deleted
  VARIANT 7: note = L, I, or V
  VARIANT 5: note = I, Y, Q, N, L, or F
XYKGXTXXXXX

SEQ ID NO: 157 - protein, 11 aa, synthetic construct
  VARIANT 1: note = G or A
  VARIANT 8: note = A, G, or V
  VARIANT 9: note = K, N, or Q
  VARIANT 10: note = W or F
  VARIANT 11: note = M, M-NH2, L, I, V, A, or G
  VARIANT 1: note = may be deleted
  VARIANT 8..11: note = may be deleted
  VARIANT 9..11: note = may be deleted
  VARIANT 10..11: note = may be deleted
  VARIANT 11: note = may be deleted
  VARIANT 7..11: note = may be deleted
  VARIANT 7: note = L, I, or V
  VARIANT 4: note = G or A
XYKXISXXXXX

SEQ ID NO: 158 - protein, 11 aa, synthetic construct
  VARIANT 1: note = G or A
  VARIANT 8: note = A, G, or V
  VARIANT 9: note = K, N, or Q
  VARIANT 10: note = W or F
  VARIANT 11: note = M, M-NH2, L, I, V, A, or G
  VARIANT 1: note = may be deleted
  VARIANT 8..11: note = may be deleted
  VARIANT 9..11: note = may be deleted
  VARIANT 10..11: note = may be deleted
  VARIANT 11: note = may be deleted
  VARIANT 7..11: note = may be deleted
  VARIANT 7: note = L, I, or V
  VARIANT 4: note = G or A
XYKXITXXXXX

SEQ ID NO: 159 - protein, 11 aa, synthetic construct
  VARIANT 1: note = G or A
  VARIANT 8: note = A, G, or V
  VARIANT 9: note = K, N, or Q
  VARIANT 10: note = W or F
  VARIANT 11: note = M, M-NH2, L, I, V, A, or G
  VARIANT 1: note = may be deleted
  VARIANT 8..11: note = may be deleted
  VARIANT 9..11: note = may be deleted
  VARIANT 10..11: note = may be deleted
  VARIANT 11: note = may be deleted
  VARIANT 7..11: note = may be deleted
  VARIANT 7: note = L, I, or V
  VARIANT 4: note = G or A
XYKXYSXXXXX

SEQ ID NO: 160 - protein, 11 aa, synthetic construct
  VARIANT 1: note = G or A
  VARIANT 8: note = A, G, or V
  VARIANT 9: note = K, N, or Q
  VARIANT 10: note = W or F
  VARIANT 11: note = M, M-NH2, L, I, V, A, or G
  VARIANT 1: note = may be deleted
  VARIANT 8..11: note = may be deleted
  VARIANT 9..11: note = may be deleted
  VARIANT 10..11: note = may be deleted
  VARIANT 11: note = may be deleted
  VARIANT 7..11: note = may be deleted
  VARIANT 7: note = L, I, or V
  VARIANT 4: note = G or A
XYKXYTXXXXX

SEQ ID NO: 161 - protein, 11 aa, synthetic construct
  VARIANT 1: note = G or A
  VARIANT 8: note = A, G, or V
  VARIANT 9: note = K, N, or Q
  VARIANT 10: note = W or F
  VARIANT 11: note = M, M-NH2, L, I, V, A, or G
  VARIANT 1: note = may be deleted
  VARIANT 8..11: note = may be deleted
  VARIANT 9..11: note = may be deleted
  VARIANT 10..11: note = may be deleted
  VARIANT 11: note = may be deleted
  VARIANT 7..11: note = may be deleted
  VARIANT 7: note = L, I, or V
XYKGYSXXXXX

SEQ ID NO: 162 - protein, 11 aa, synthetic construct
  VARIANT 1: note = G or A
  VARIANT 8: note = A, G, or V
  VARIANT 9: note = K, N, or Q
  VARIANT 10: note = W or F
  VARIANT 11: note = M, M-NH2, L, I, V, A, or G
  VARIANT 1: note = may be deleted
  VARIANT 8..11: note = may be deleted
  VARIANT 9..11: note = may be deleted
  VARIANT 10..11: note = may be deleted
  VARIANT 11: note = may be deleted
  VARIANT 7..11: note = may be deleted
  VARIANT 7: note = L, I, or V
XYKGISXXXXX

SEQ ID NO: 163 - protein, 11 aa, synthetic construct
  VARIANT 1: note = G or A
  VARIANT 8: note = A, G, or V
  VARIANT 9: note = K, N, or Q
  VARIANT 10: note = W or F
  VARIANT 11: note = M, M-NH2, L, I, V, A, or G
  VARIANT 1: note = may be deleted
  VARIANT 8..11: note = may be deleted
  VARIANT 9..11: note = may be deleted
  VARIANT 10..11: note = may be deleted
  VARIANT 11: note = may be deleted
  VARIANT 7..11: note = may be deleted
  VARIANT 7: note = L, I, or V
XYKGYTXXXXX

SEQ ID NO: 164 - protein, 11 aa, synthetic construct
  VARIANT 1: note = G or A
  VARIANT 8: note = A, G, or V
  VARIANT 9: note = K, N, or Q
  VARIANT 10: note = W or F
  VARIANT 11: note = M, M-NH2, L, I, V, A, or G
  VARIANT 1: note = may be deleted
  VARIANT 8..11: note = may be deleted
  VARIANT 9..11: note = may be deleted
  VARIANT 10..11: note = may be deleted
  VARIANT 11: note = may be deleted
  VARIANT 7..11: note = may be deleted
  VARIANT 7: note = L, I, or V
XYKGITXXXXX

SEQ ID NO: 165 - protein, 11 aa, synthetic construct
  VARIANT 1: note = G or A
  VARIANT 8: note = A, G, or V
  VARIANT 9: note = K, N, or Q
  VARIANT 10: note = W or F
  VARIANT 11: note = M, M-NH2, L, I, V, A, or G
  VARIANT 1: note = may be deleted
  VARIANT 8..11: note = may be deleted
  VARIANT 9..11: note = may be deleted
  VARIANT 10..11: note = may be deleted
  VARIANT 11: note = may be deleted
  VARIANT 7..11: note = may be deleted
  VARIANT 7: note = L, I, or V
  VARIANT 6: note = S or T
XYLGIXXXXXX

SEQ ID NO: 166 - protein, 11 aa, synthetic construct
  VARIANT 1: note = G or A
  VARIANT 8: note = A, G, or V
  VARIANT 9: note = K, N, or Q
  VARIANT 10: note = W or F
  VARIANT 11: note = M, M-NH2, L, I, V, A, or G
  VARIANT 1: note = may be deleted
  VARIANT 8..11: note = may be deleted
  VARIANT 9..11: note = may be deleted
  VARIANT 10..11: note = may be deleted
  VARIANT 11: note = may be deleted
  VARIANT 7..11: note = may be deleted
  VARIANT 7: note = L, I, or V
  VARIANT 6: note = S or T
XYLGYXXXXXX

SEQ ID NO: 167 - protein, 11 aa, synthetic construct
  VARIANT 1: note = G or A
  VARIANT 8: note = A, G, or V
  VARIANT 9: note = K, N, or Q
  VARIANT 10: note = W or F
  VARIANT 11: note = M, M-NH2, L, I, V, A, or G
  VARIANT 1: note = may be deleted
  VARIANT 8..11: note = may be deleted
  VARIANT 9..11: note = may be deleted
  VARIANT 10..11: note = may be deleted
  VARIANT 11: note = may be deleted
  VARIANT 7..11: note = may be deleted
  VARIANT 7: note = L, I, or V
  VARIANT 5: note = I, Y, Q, N, L, or F
XYLGXSXXXXX

SEQ ID NO: 168 - protein, 11 aa, synthetic construct
  VARIANT 1: note = G or A
  VARIANT 8: note = A, G, or V
  VARIANT 9: note = K, N, or Q
  VARIANT 10: note = W or F
  VARIANT 11: note = M, M-NH2, L, I, V, A, or G
  VARIANT 1: note = may be deleted
  VARIANT 8..11: note = may be deleted
  VARIANT 9..11: note = may be deleted
  VARIANT 10..11: note = may be deleted
  VARIANT 11: note = may be deleted
  VARIANT 7..11: note = may be deleted
  VARIANT 7: note = L, I, or V
  VARIANT 5: note = I, Y, Q, N, L, or F
XYLGXTXXXXX

SEQ ID NO: 169 - protein, 11 aa, synthetic construct
  VARIANT 1: note = G or A
  VARIANT 8: note = A, G, or V
  VARIANT 9: note = K, N, or Q
  VARIANT 10: note = W or F
  VARIANT 11: note = M, M-NH2, L, I, V, A, or G
  VARIANT 1: note = may be deleted
  VARIANT 8..11: note = may be deleted
  VARIANT 9..11: note = may be deleted
  VARIANT 10..11: note = may be deleted
  VARIANT 11: note = may be deleted
  VARIANT 7..11: note = may be deleted
  VARIANT 7: note = L, I, or V
  VARIANT 4: note = G or A
XYLXISXXXXX

SEQ ID NO: 170 - protein, 11 aa, synthetic construct
  VARIANT 1: note = G or A
  VARIANT 8: note = A, G, or V
  VARIANT 9: note = K, N, or Q
  VARIANT 10: note = W or F
  VARIANT 11: note = M, M-NH2, L, I, V, A, or G
  VARIANT 1: note = may be deleted
  VARIANT 8..11: note = may be deleted
  VARIANT 9..11: note = may be deleted
  VARIANT 10..11: note = may be deleted
  VARIANT 11: note = may be deleted
  VARIANT 7..11: note = may be deleted
  VARIANT 7: note = L, I, or V
  VARIANT 4: note = G or A
XYLXITXXXXX

SEQ ID NO: 171 - protein, 11 aa, synthetic construct
  VARIANT 1: note = G or A
  VARIANT 8: note = A, G, or V
  VARIANT 9: note = K, N, or Q
  VARIANT 10: note = W or F
  VARIANT 11: note = M, M-NH2, L, I, V, A, or G
  VARIANT 1: note = may be deleted
  VARIANT 8..11: note = may be deleted
  VARIANT 9..11: note = may be deleted
  VARIANT 10..11: note = may be deleted
  VARIANT 11: note = may be deleted
  VARIANT 7..11: note = may be deleted
  VARIANT 7: note = L, I, or V
  VARIANT 4: note = G or A
XYLXYSXXXXX

SEQ ID NO: 172 - protein, 11 aa, synthetic construct
  VARIANT 1: note = G or A
  VARIANT 8: note = A, G, or V
  VARIANT 9: note = K, N, or Q
  VARIANT 10: note = W or F
  VARIANT 11: note = M, M-NH2, L, I, V, A, or G
  VARIANT 1: note = may be deleted
  VARIANT 8..11: note = may be deleted
  VARIANT 9..11: note = may be deleted
  VARIANT 10..11: note = may be deleted
  VARIANT 11: note = may be deleted
  VARIANT 7..11: note = may be deleted
  VARIANT 7: note = L, I, or V
  VARIANT 4: note = G or A
XYLXYTXXXXX

SEQ ID NO: 173 - protein, 11 aa, synthetic construct
  VARIANT 1: note = G or A
  VARIANT 8: note = A, G, or V
  VARIANT 9: note = K, N, or Q
  VARIANT 10: note = W or F
  VARIANT 11: note = M, M-NH2, L, I, V, A, or G
  VARIANT 1: note = may be deleted
  VARIANT 8..11: note = may be deleted
  VARIANT 9..11: note = may be deleted
  VARIANT 10..11: note = may be deleted
  VARIANT 11: note = may be deleted
  VARIANT 7..11: note = may be deleted
  VARIANT 7: note = L, I, or V
XYLGYSXXXXX

SEQ ID NO: 174 - protein, 11 aa, synthetic construct
  VARIANT 1: note = G or A
  VARIANT 8: note = A, G, or V
  VARIANT 9: note = K, N, or Q
  VARIANT 10: note = W or F
  VARIANT 11: note = M, M-NH2, L, I, V, A, or G
  VARIANT 1: note = may be deleted
  VARIANT 8..11: note = may be deleted
  VARIANT 9..11: note = may be deleted
  VARIANT 10..11: note = may be deleted
  VARIANT 11: note = may be deleted
  VARIANT 7..11: note = may be deleted
  VARIANT 7: note = L, I, or V
XYLGISXXXXX

SEQ ID NO: 175 - protein, 11 aa, synthetic construct
  VARIANT 1: note = G or A
  VARIANT 8: note = A, G, or V
  VARIANT 9: note = K, N, or Q
  VARIANT 10: note = W or F
  VARIANT 11: note = M, M-NH2, L, I, V, A, or G
  VARIANT 1: note = may be deleted
  VARIANT 8..11: note = may be deleted
  VARIANT 9..11: note = may be deleted
  VARIANT 10..11: note = may be deleted
  VARIANT 11: note = may be deleted
  VARIANT 7..11: note = may be deleted
  VARIANT 7: note = L, I, or V
XYLGYTXXXXX

SEQ ID NO: 176 - protein, 11 aa, synthetic construct
  VARIANT 1: note = G or A
  VARIANT 8: note = A, G, or V
  VARIANT 9: note = K, N, or Q
  VARIANT 10: note = W or F
  VARIANT 11: note = M, M-NH2, L, I, V, A, or G
  VARIANT 1: note = may be deleted
  VARIANT 8..11: note = may be deleted
  VARIANT 9..11: note = may be deleted
  VARIANT 10..11: note = may be deleted
  VARIANT 11: note = may be deleted
  VARIANT 7..11: note = may be deleted
  VARIANT 7: note = L, I, or V
XYLGITXXXXX

SEQ ID NO: 177 - protein, 11 aa, synthetic construct
  VARIANT 1: note = G or A
  VARIANT 8: note = A, G, or V
  VARIANT 9: note = K, N, or Q
  VARIANT 10: note = W or F
  VARIANT 11: note = M, M-NH2, L, I, V, A, or G
  VARIANT 1: note = may be deleted
  VARIANT 8..11: note = may be deleted
  VARIANT 9..11: note = may be deleted
  VARIANT 10..11: note = may be deleted
  VARIANT 11: note = may be deleted
  VARIANT 7..11: note = may be deleted
  VARIANT 7: note = L, I, or V
  VARIANT 6: note = S or T
XFRGIXXXXXX

SEQ ID NO: 178 - protein, 11 aa, synthetic construct
  VARIANT 1: note = G or A
  VARIANT 8: note = A, G, or V
  VARIANT 9: note = K, N, or Q
  VARIANT 10: note = W or F
  VARIANT 11: note = M, M-NH2, L, I, V, A, or G
  VARIANT 1: note = may be deleted
  VARIANT 8..11: note = may be deleted
  VARIANT 9..11: note = may be deleted
  VARIANT 10..11: note = may be deleted
  VARIANT 11: note = may be deleted
  VARIANT 7..11: note = may be deleted
  VARIANT 7: note = L, I, or V
  VARIANT 6: note = S or T
XFRGYXXXXXX

SEQ ID NO: 179 - protein, 11 aa, synthetic construct
  VARIANT 1: note = G or A
  VARIANT 8: note = A, G, or V
  VARIANT 9: note = K, N, or Q
  VARIANT 10: note = W or F
  VARIANT 11: note = M, M-NH2, L, I, V, A, or G
  VARIANT 1: note = may be deleted
  VARIANT 8..11: note = may be deleted
  VARIANT 9..11: note = may be deleted
  VARIANT 10..11: note = may be deleted
  VARIANT 11: note = may be deleted
  VARIANT 7..11: note = may be deleted
  VARIANT 7: note = L, I, or V
  VARIANT 5: note = I, Y, Q, N, L, or F
XFRGXSXXXXX

SEQ ID NO: 180 - protein, 11 aa, synthetic construct
  VARIANT 1: note = G or A
  VARIANT 8: note = A, G, or V
  VARIANT 9: note = K, N, or Q
  VARIANT 10: note = W or F
  VARIANT 11: note = M, M-NH2, L, I, V, A, or G
  VARIANT 1: note = may be deleted
  VARIANT 8..11: note = may be deleted
  VARIANT 9..11: note = may be deleted
  VARIANT 10..11: note = may be deleted
  VARIANT 11: note = may be deleted
  VARIANT 7..11: note = may be deleted
  VARIANT 7: note = L, I, or V
  VARIANT 5: note = I, Y, Q, N, L, or F
XFRGXTXXXXX

SEQ ID NO: 181 - protein, 11 aa, synthetic construct
  VARIANT 1: note = G or A
  VARIANT 8: note = A, G, or V
  VARIANT 9: note = K, N, or Q
  VARIANT 10: note = W or F
  VARIANT 11: note = M, M-NH2, L, I, V, A, or G
  VARIANT 1: note = may be deleted
  VARIANT 8..11: note = may be deleted
  VARIANT 9..11: note = may be deleted
  VARIANT 10..11: note = may be deleted
  VARIANT 11: note = may be deleted
  VARIANT 7..11: note = may be deleted
  VARIANT 7: note = L, I, or V
  VARIANT 4: note = G or A
XFRXISXXXXX

SEQ ID NO: 182 - protein, 11 aa, synthetic construct
  VARIANT 1: note = G or A
  VARIANT 8: note = A, G, or V
  VARIANT 9: note = K, N, or Q
  VARIANT 10: note = W or F
  VARIANT 11: note = M, M-NH2, L, I, V, A, or G
  VARIANT 1: note = may be deleted
  VARIANT 8..11: note = may be deleted
  VARIANT 9..11: note = may be deleted
  VARIANT 10..11: note = may be deleted
  VARIANT 11: note = may be deleted
  VARIANT 7..11: note = may be deleted
  VARIANT 7: note = L, I, or V
  VARIANT 4: note = G or A
XFRXITXXXXX

SEQ ID NO: 183 - protein, 11 aa, synthetic construct
  VARIANT 1: note = G or A
  VARIANT 8: note = A, G, or V
  VARIANT 9: note = K, N, or Q
  VARIANT 10: note = W or F
  VARIANT 11: note = M, M-NH2, L, I, V, A, or G
  VARIANT 1: note = may be deleted
  VARIANT 8..11: note = may be deleted
  VARIANT 9..11: note = may be deleted
  VARIANT 10..11: note = may be deleted
  VARIANT 11: note = may be deleted
  VARIANT 7..11: note = may be deleted
  VARIANT 7: note = L, I, or V
  VARIANT 4: note = G or A
XFRXYSXXXXX

SEQ ID NO: 184 - protein, 11 aa, synthetic construct
  VARIANT 1: note = G or A
  VARIANT 8: note = A, G, or V
  VARIANT 9: note = K, N, or Q
  VARIANT 10: note = W or F
  VARIANT 11: note = M, M-NH2, L, I, V, A, or G
  VARIANT 1: note = may be deleted
  VARIANT 8..11: note = may be deleted
  VARIANT 9..11: note = may be deleted
  VARIANT 10..11: note = may be deleted
  VARIANT 11: note = may be deleted
  VARIANT 7..11: note = may be deleted
  VARIANT 7: note = L, I, or V
  VARIANT 4: note = G or A
XFRXYTXXXXX

SEQ ID NO: 185 - protein, 11 aa, synthetic construct
  VARIANT 1: note = G or A
  VARIANT 8: note = A, G, or V
  VARIANT 9: note = K, N, or Q
  VARIANT 10: note = W or F
  VARIANT 11: note = M, M-NH2, L, I, V, A, or G
  VARIANT 1: note = may be deleted
  VARIANT 8..11: note = may be deleted
  VARIANT 9..11: note = may be deleted
  VARIANT 10..11: note = may be deleted
  VARIANT 11: note = may be deleted
  VARIANT 7..11: note = may be deleted
  VARIANT 7: note = L, I, or V
XFRGYSXXXXX

SEQ ID NO: 186 - protein, 11 aa, synthetic construct
  VARIANT 1: note = G or A
  VARIANT 8: note = A, G, or V
  VARIANT 9: note = K, N, or Q
  VARIANT 10: note = W or F
  VARIANT 11: note = M, M-NH2, L, I, V, A, or G
  VARIANT 1: note = may be deleted
  VARIANT 8..11: note = may be deleted
  VARIANT 9..11: note = may be deleted
  VARIANT 10..11: note = may be deleted
  VARIANT 11: note = may be deleted
  VARIANT 7..11: note = may be deleted
  VARIANT 7: note = L, I, or V
XFRGISXXXXX

SEQ ID NO: 187 - protein, 11 aa, synthetic construct
  VARIANT 1: note = G or A
  VARIANT 8: note = A, G, or V
  VARIANT 9: note = K, N, or Q
  VARIANT 10: note = W or F
  VARIANT 11: note = M, M-NH2, L, I, V, A, or G
  VARIANT 1: note = may be deleted
  VARIANT 8..11: note = may be deleted
  VARIANT 9..11: note = may be deleted
  VARIANT 10..11: note = may be deleted
  VARIANT 11: note = may be deleted
  VARIANT 7..11: note = may be deleted
  VARIANT 7: note = L, I, or V
XFRGYTXXXXX

SEQ ID NO: 188 - protein, 11 aa, synthetic construct
  VARIANT 1: note = G or A
  VARIANT 8: note = A, G, or V
  VARIANT 9: note = K, N, or Q
  VARIANT 10: note = W or F
  VARIANT 11: note = M, M-NH2, L, I, V, A, or G
  VARIANT 1: note = may be deleted
  VARIANT 8..11: note = may be deleted
  VARIANT 9..11: note = may be deleted
  VARIANT 10..11: note = may be deleted
  VARIANT 11: note = may be deleted
  VARIANT 7..11: note = may be deleted
  VARIANT 7: note = L, I, or V
XFRGITXXXXX

SEQ ID NO: 189 - protein, 11 aa, synthetic construct
  VARIANT 1: note = G or A
  VARIANT 8: note = A, G, or V
  VARIANT 9: note = K, N, or Q
  VARIANT 10: note = W or F
  VARIANT 11: note = M, M-NH2, L, I, V, A, or G
  VARIANT 1: note = may be deleted
  VARIANT 8..11: note = may be deleted
  VARIANT 9..11: note = may be deleted
  VARIANT 10..11: note = may be deleted
  VARIANT 11: note = may be deleted
  VARIANT 7..11: note = may be deleted
  VARIANT 7: note = L, I, or V
  VARIANT 6: note = S or T
XFKGIXXXXXX

SEQ ID NO: 190 - protein, 11 aa, synthetic construct
  VARIANT 1: note = G or A
  VARIANT 8: note = A, G, or V
  VARIANT 9: note = K, N, or Q
  VARIANT 10: note = W or F
  VARIANT 11: note = M, M-NH2, L, I, V, A, or G
  VARIANT 1: note = may be deleted
  VARIANT 8..11: note = may be deleted
  VARIANT 9..11: note = may be deleted
  VARIANT 10..11: note = may be deleted
  VARIANT 11: note = may be deleted
  VARIANT 7..11: note = may be deleted
  VARIANT 7: note = L, I, or V
  VARIANT 6: note = S or T
XFKGYXXXXXX

SEQ ID NO: 191 - protein, 11 aa, synthetic construct
  VARIANT 1: note = G or A
  VARIANT 8: note = A, G, or V
  VARIANT 9: note = K, N, or Q
  VARIANT 10: note = W or F
  VARIANT 11: note = M, M-NH2, L, I, V, A, or G
  VARIANT 1: note = may be deleted
  VARIANT 8..11: note = may be deleted
  VARIANT 9..11: note = may be deleted
  VARIANT 10..11: note = may be deleted
  VARIANT 11: note = may be deleted
  VARIANT 7..11: note = may be deleted
  VARIANT 7: note = L, I, or V
  VARIANT 5: note = I, Y, Q, N, L, or F
XFKGXSXXXXX

SEQ ID NO: 192 - protein, 11 aa, synthetic construct
  VARIANT 1: note = G or A
  VARIANT 8: note = A, G, or V
  VARIANT 9: note = K, N, or Q
  VARIANT 10: note = W or F
  VARIANT 11: note = M, M-NH2, L, I, V, A, or G
  VARIANT 1: note = may be deleted
  VARIANT 8..11: note = may be deleted
  VARIANT 9..11: note = may be deleted
  VARIANT 10..11: note = may be deleted
  VARIANT 11: note = may be deleted
  VARIANT 7..11: note = may be deleted
  VARIANT 7: note = L, I, or V
  VARIANT 5: note = I, Y, Q, N, L, or F
XFKGXTXXXXX

SEQ ID NO: 193 - protein, 11 aa, synthetic construct
  VARIANT 1: note = G or A
  VARIANT 8: note = A, G, or V
  VARIANT 9: note = K, N, or Q
  VARIANT 10: note = W or F
  VARIANT 11: note = M, M-NH2, L, I, V, A, or G
  VARIANT 1: note = may be deleted
  VARIANT 8..11: note = may be deleted
  VARIANT 9..11: note = may be deleted
  VARIANT 10..11: note = may be deleted
  VARIANT 11: note = may be deleted
  VARIANT 7..11: note = may be deleted
  VARIANT 7: note = L, I, or V
  VARIANT 4: note = G or A
XFKXISXXXXX

SEQ ID NO: 194 - protein, 11 aa, synthetic construct
  VARIANT 1: note = G or A
  VARIANT 8: note = A, G, or V
  VARIANT 9: note = K, N, or Q
  VARIANT 10: note = W or F
  VARIANT 11: note = M, M-NH2, L, I, V, A, or G
  VARIANT 1: note = may be deleted
  VARIANT 8..11: note = may be deleted
  VARIANT 9..11: note = may be deleted
  VARIANT 10..11: note = may be deleted
  VARIANT 11: note = may be deleted
  VARIANT 7..11: note = may be deleted
  VARIANT 7: note = L, I, or V
  VARIANT 4: note = G or A
XFKXITXXXXX

SEQ ID NO: 195 - protein, 11 aa, synthetic construct
  VARIANT 1: note = G or A
  VARIANT 8: note = A, G, or V
  VARIANT 9: note = K, N, or Q
  VARIANT 10: note = W or F
  VARIANT 11: note = M, M-NH2, L, I, V, A, or G
  VARIANT 1: note = may be deleted
  VARIANT 8..11: note = may be deleted
  VARIANT 9..11: note = may be deleted
  VARIANT 10..11: note = may be deleted
  VARIANT 11: note = may be deleted
  VARIANT 7..11: note = may be deleted
  VARIANT 7: note = L, I, or V
  VARIANT 4: note = G or A
XFKXYSXXXXX

SEQ ID NO: 196 - protein, 11 aa, synthetic construct
  VARIANT 1: note = G or A
  VARIANT 8: note = A, G, or V
  VARIANT 9: note = K, N, or Q
  VARIANT 10: note = W or F
  VARIANT 11: note = M, M-NH2, L, I, V, A, or G
  VARIANT 1: note = may be deleted
  VARIANT 8..11: note = may be deleted
  VARIANT 9..11: note = may be deleted
  VARIANT 10..11: note = may be deleted
  VARIANT 11: note = may be deleted
  VARIANT 7..11: note = may be deleted
  VARIANT 7: note = L, I, or V
  VARIANT 4: note = G or A
XFKXYTXXXXX

SEQ ID NO: 197 - protein, 11 aa, synthetic construct
  VARIANT 1: note = G or A
  VARIANT 8: note = A, G, or V
  VARIANT 9: note = K, N, or Q
  VARIANT 10: note = W or F
  VARIANT 11: note = M, M-NH2, L, I, V, A, or G
  VARIANT 1: note = may be deleted
  VARIANT 8..11: note = may be deleted
  VARIANT 9..11: note = may be deleted
  VARIANT 10..11: note = may be deleted
  VARIANT 11: note = may be deleted
  VARIANT 7..11: note = may be deleted
  VARIANT 7: note = L, I, or V
XFKGYSXXXXX

SEQ ID NO: 198 - protein, 11 aa, synthetic construct
  VARIANT 1: note = G or A
  VARIANT 8: note = A, G, or V
  VARIANT 9: note = K, N, or Q
  VARIANT 10: note = W or F
  VARIANT 11: note = M, M-NH2, L, I, V, A, or G
  VARIANT 1: note = may be deleted
  VARIANT 8..11: note = may be deleted
  VARIANT 9..11: note = may be deleted
  VARIANT 10..11: note = may be deleted
  VARIANT 11: note = may be deleted
  VARIANT 7..11: note = may be deleted
  VARIANT 7: note = L, I, or V
XFKGISXXXXX

SEQ ID NO: 199 - protein, 11 aa, synthetic construct
  VARIANT 1: note = G or A
  VARIANT 8: note = A, G, or V
  VARIANT 9: note = K, N, or Q
  VARIANT 10: note = W or F
  VARIANT 11: note = M, M-NH2, L, I, V, A, or G
  VARIANT 1: note = may be deleted
  VARIANT 8..11: note = may be deleted
  VARIANT 9..11: note = may be deleted
  VARIANT 10..11: note = may be deleted
  VARIANT 11: note = may be deleted
  VARIANT 7..11: note = may be deleted
  VARIANT 7: note = L, I, or V
XFKGYTXXXXX

SEQ ID NO: 200 - protein, 11 aa, synthetic construct
  VARIANT 1: note = G or A
  VARIANT 8: note = A, G, or V
  VARIANT 9: note = K, N, or Q
  VARIANT 10: note = W or F
  VARIANT 11: note = M, M-NH2, L, I, V, A, or G
  VARIANT 1: note = may be deleted
  VARIANT 8..11: note = may be deleted
  VARIANT 9..11: note = may be deleted
  VARIANT 10..11: note = may be deleted
  VARIANT 11: note = may be deleted
  VARIANT 7..11: note = may be deleted
  VARIANT 7: note = L, I, or V
XFKGITXXXXX

SEQ ID NO: 201 - protein, 11 aa, synthetic construct
  VARIANT 1: note = G or A
  VARIANT 8: note = A, G, or V
  VARIANT 9: note = K, N, or Q
  VARIANT 10: note = W or F
  VARIANT 11: note = M, M-NH2, L, I, V, A, or G
  VARIANT 1: note = may be deleted
  VARIANT 8..11: note = may be deleted
  VARIANT 9..11: note = may be deleted
  VARIANT 10..11: note = may be deleted
  VARIANT 11: note = may be deleted
  VARIANT 7..11: note = may be deleted
  VARIANT 7: note = L, I, or V
  VARIANT 6: note = S or T
XFLGYXXXXXX

SEQ ID NO: 202 - protein, 11 aa, synthetic construct
  VARIANT 1: note = G or A
  VARIANT 8: note = A, G, or V
  VARIANT 9: note = K, N, or Q
  VARIANT 10: note = W or F
  VARIANT 11: note = M, M-NH2, L, I, V, A, or G
  VARIANT 1: note = may be deleted
  VARIANT 8..11: note = may be deleted
  VARIANT 9..11: note = may be deleted
  VARIANT 10..11: note = may be deleted
  VARIANT 11: note = may be deleted
  VARIANT 7..11: note = may be deleted
  VARIANT 7: note = L, I, or V
  VARIANT 5: note = I, Y, Q, N, L, or F
XFLGXSXXXXX

SEQ ID NO: 203 - protein, 11 aa, synthetic construct
  VARIANT 1: note = G or A
  VARIANT 8: note = A, G, or V
  VARIANT 9: note = K, N, or Q
  VARIANT 10: note = W or F
  VARIANT 11: note = M, M-NH2, L, I, V, A, or G
  VARIANT 1: note = may be deleted
  VARIANT 8..11: note = may be deleted
  VARIANT 9..11: note = may be deleted
  VARIANT 10..11: note = may be deleted
  VARIANT 11: note = may be deleted
  VARIANT 7..11: note = may be deleted
  VARIANT 7: note = L, I, or V
  VARIANT 5: note = I, Y, Q, N, L, or F
XFLGXTXXXXX

SEQ ID NO: 204 - protein, 11 aa, synthetic construct
  VARIANT 1: note = G or A
  VARIANT 8: note = A, G, or V
  VARIANT 9: note = K, N, or Q
  VARIANT 10: note = W or F
  VARIANT 11: note = M, M-NH2, L, I, V, A, or G
  VARIANT 1: note = may be deleted
  VARIANT 8..11: note = may be deleted
  VARIANT 9..11: note = may be deleted
  VARIANT 10..11: note = may be deleted
  VARIANT 11: note = may be deleted
  VARIANT 7..11: note = may be deleted
  VARIANT 7: note = L, I, or V
  VARIANT 4: note = G or A
XFLXISXXXXX

SEQ ID NO: 205 - protein, 11 aa, synthetic construct
  VARIANT 1: note = G or A
  VARIANT 8: note = A, G, or V
  VARIANT 9: note = K, N, or Q
  VARIANT 10: note = W or F
  VARIANT 11: note = M, M-NH2, L, I, V, A, or G
  VARIANT 1: note = may be deleted
  VARIANT 8..11: note = may be deleted
  VARIANT 9..11: note = may be deleted
  VARIANT 10..11: note = may be deleted
  VARIANT 11: note = may be deleted
  VARIANT 7..11: note = may be deleted
  VARIANT 7: note = L, I, or V
  VARIANT 4: note = G or A
XFLXITXXXXX

SEQ ID NO: 206 - protein, 11 aa, synthetic construct
  VARIANT 1: note = G or A
  VARIANT 8: note = A, G, or V
  VARIANT 9: note = K, N, or Q
  VARIANT 10: note = W or F
  VARIANT 11: note = M, M-NH2, L, I, V, A, or G
  VARIANT 1: note = may be deleted
  VARIANT 8..11: note = may be deleted
  VARIANT 9..11: note = may be deleted
  VARIANT 10..11: note = may be deleted
  VARIANT 11: note = may be deleted
  VARIANT 7..11: note = may be deleted
  VARIANT 7: note = L, I, or V
  VARIANT 4: note = G or A
XFLXYSXXXXX

SEQ ID NO: 207 - protein, 11 aa, synthetic construct
  VARIANT 1: note = G or A
  VARIANT 8: note = A, G, or V
  VARIANT 9: note = K, N, or Q
  VARIANT 10: note = W or F
  VARIANT 11: note = M, M-NH2, L, I, V, A, or G
  VARIANT 1: note = may be deleted
  VARIANT 8..11: note = may be deleted
  VARIANT 9..11: note = may be deleted
  VARIANT 10..11: note = may be deleted
  VARIANT 11: note = may be deleted
  VARIANT 7..11: note = may be deleted
  VARIANT 7: note = L, I, or V
  VARIANT 4: note = G or A
XFLXYTXXXXX

SEQ ID NO: 208 - protein, 11 aa, synthetic construct
  VARIANT 1: note = G or A
  VARIANT 8: note = A, G, or V
  VARIANT 9: note = K, N, or Q
  VARIANT 10: note = W or F
  VARIANT 11: note = M, M-NH2, L, I, V, A, or G
  VARIANT 1: note = may be deleted
  VARIANT 8..11: note = may be deleted
  VARIANT 9..11: note = may be deleted
  VARIANT 10..11: note = may be deleted
  VARIANT 11: note = may be deleted
  VARIANT 7..11: note = may be deleted
  VARIANT 7: note = L, I, or V
XFLGYSXXXXX

SEQ ID NO: 209 - protein, 11 aa, synthetic construct
  VARIANT 1: note = G or A
  VARIANT 8: note = A, G, or V
  VARIANT 9: note = K, N, or Q
  VARIANT 10: note = W or F
  VARIANT 11: note = M, M-NH2, L, I, V, A, or G
  VARIANT 1: note = may be deleted
  VARIANT 8..11: note = may be deleted
  VARIANT 9..11: note = may be deleted
  VARIANT 10..11: note = may be deleted
  VARIANT 11: note = may be deleted
  VARIANT 7..11: note = may be deleted
  VARIANT 7: note = L, I, or V
XFLGISXXXXX

SEQ ID NO: 210 - protein, 11 aa, synthetic construct
  VARIANT 1: note = G or A
  VARIANT 8: note = A, G, or V
  VARIANT 9: note = K, N, or Q
  VARIANT 10: note = W or F
  VARIANT 11: note = M, M-NH2, L, I, V, A, or G
  VARIANT 1: note = may be deleted
  VARIANT 8..11: note = may be deleted
  VARIANT 9..11: note = may be deleted
  VARIANT 10..11: note = may be deleted
  VARIANT 11: note = may be deleted
  VARIANT 7..11: note = may be deleted
  VARIANT 7: note = L, I, or V
XFLGYTXXXXX

SEQ ID NO: 211 - protein, 11 aa, synthetic construct
  VARIANT 1: note = G or A
  VARIANT 8: note = A, G, or V
  VARIANT 9: note = K, N, or Q
  VARIANT 10: note = W or F
  VARIANT 11: note = M, M-NH2, L, I, V, A, or G
  VARIANT 1: note = may be deleted
  VARIANT 8..11: note = may be deleted
  VARIANT 9..11: note = may be deleted
  VARIANT 10..11: note = may be deleted
  VARIANT 11: note = may be deleted
  VARIANT 7..11: note = may be deleted
  VARIANT 7: note = L, I, or V
XFLGITXXXXX

SEQ ID NO: 212 - protein, 11 aa, synthetic construct
  VARIANT 8: note = A, G, or V
  VARIANT 9: note = K, N, or Q
  VARIANT 10: note = W or F
  VARIANT 11: note = M, M-NH2, L, I, V, A, or G
  VARIANT 8..11: note = may be deleted
  VARIANT 9..11: note = may be deleted
  VARIANT 10..11: note = may be deleted
  VARIANT 11: note = may be deleted
  VARIANT 7..11: note = may be deleted
  VARIANT 7: note = L, I, or V
  VARIANT 6: note = S or T
GYRGIXXXXXX

SEQ ID NO: 213 - protein, 11 aa, synthetic construct
  VARIANT 8: note = A, G, or V
  VARIANT 9: note = K, N, or Q
  VARIANT 10: note = W or F
  VARIANT 11: note = M, M-NH2, L, I, V, A, or G
  VARIANT 8..11: note = may be deleted
  VARIANT 9..11: note = may be deleted
  VARIANT 10..11: note = may be deleted
  VARIANT 11: note = may be deleted
  VARIANT 7..11: note = may be deleted
  VARIANT 7: note = L, I, or V
  VARIANT 6: note = S or T
GYRGYXXXXXX

SEQ ID NO: 214 - protein, 11 aa, synthetic construct
  VARIANT 8: note = A, G, or V
  VARIANT 9: note = K, N, or Q
  VARIANT 10: note = W or F
  VARIANT 11: note = M, M-NH2, L, I, V, A, or G
  VARIANT 8..11: note = may be deleted
  VARIANT 9..11: note = may be deleted
  VARIANT 10..11: note = may be deleted
  VARIANT 11: note = may be deleted
  VARIANT 7..11: note = may be deleted
  VARIANT 7: note = L, I, or V
  VARIANT 5: note = I, Y, Q, N, L, or F
GYRGXSXXXXX

SEQ ID NO: 215 - protein, 11 aa, synthetic construct
  VARIANT 8: note = A, G, or V
  VARIANT 9: note = K, N, or Q
  VARIANT 10: note = W or F
  VARIANT 11: note = M, M-NH2, L, I, V, A, or G
  VARIANT 8..11: note = may be deleted
  VARIANT 9..11: note = may be deleted
  VARIANT 10..11: note = may be deleted
  VARIANT 11: note = may be deleted
  VARIANT 7..11: note = may be deleted
  VARIANT 7: note = L, I, or V
  VARIANT 5: note = I, Y, Q, N, L, or F
GYRGXTXXXXX

SEQ ID NO: 216 - protein, 11 aa, synthetic construct
  VARIANT 8: note = A, G, or V
  VARIANT 9: note = K, N, or Q
  VARIANT 10: note = W or F
  VARIANT 11: note = M, M-NH2, L, I, V, A, or G
  VARIANT 8..11: note = may be deleted
  VARIANT 9..11: note = may be deleted
  VARIANT 10..11: note = may be deleted
  VARIANT 11: note = may be deleted
  VARIANT 7..11: note = may be deleted
  VARIANT 7: note = L, I, or V
  VARIANT 4: note = G or A
GYRXISXXXXX

SEQ ID NO: 217 - protein, 11 aa, synthetic construct
  VARIANT 8: note = A, G, or V
  VARIANT 9: note = K, N, or Q
  VARIANT 10: note = W or F
  VARIANT 11: note = M, M-NH2, L, I, V, A, or G
  VARIANT 8..11: note = may be deleted
  VARIANT 9..11: note = may be deleted
  VARIANT 10..11: note = may be deleted
  VARIANT 11: note = may be deleted
  VARIANT 7..11: note = may be deleted
  VARIANT 7: note = L, I, or V
  VARIANT 4: note = G or A
GYRXITXXXXX

SEQ ID NO: 218 - protein, 11 aa, synthetic construct
  VARIANT 8: note = A, G, or V
  VARIANT 9: note = K, N, or Q
  VARIANT 10: note = W or F
  VARIANT 11: note = M, M-NH2, L, I, V, A, or G
  VARIANT 8..11: note = may be deleted
  VARIANT 9..11: note = may be deleted
  VARIANT 10..11: note = may be deleted
  VARIANT 11: note = may be deleted
  VARIANT 7..11: note = may be deleted
  VARIANT 7: note = L, I, or V
  VARIANT 4: note = G or A
GYRXYSXXXXX

SEQ ID NO: 219 - protein, 11 aa, synthetic construct
  VARIANT 8: note = A, G, or V
  VARIANT 9: note = K, N, or Q
  VARIANT 10: note = W or F
  VARIANT 11: note = M, M-NH2, L, I, V, A, or G
  VARIANT 8..11: note = may be deleted
  VARIANT 9..11: note = may be deleted
  VARIANT 10..11: note = may be deleted
  VARIANT 11: note = may be deleted
  VARIANT 7..11: note = may be deleted
  VARIANT 7: note = L, I, or V
  VARIANT 4: note = G or A
GYRXYTXXXXX

SEQ ID NO: 220 - protein, 11 aa, synthetic construct
  VARIANT 8: note = A, G, or V
  VARIANT 9: note = K, N, or Q
  VARIANT 10: note = W or F
  VARIANT 11: note = M, M-NH2, L, I, V, A, or G
  VARIANT 8..11: note = may be deleted
  VARIANT 9..11: note = may be deleted
  VARIANT 10..11: note = may be deleted
  VARIANT 11: note = may be deleted
  VARIANT 7..11: note = may be deleted
  VARIANT 7: note = L, I, or V
GYRGYSXXXXX

SEQ ID NO: 221 - protein, 11 aa, synthetic construct
  VARIANT 8: note = A, G, or V
  VARIANT 9: note = K, N, or Q
  VARIANT 10: note = W or F
  VARIANT 11: note = M, M-NH2, L, I, V, A, or G
  VARIANT 8..11: note = may be deleted
  VARIANT 9..11: note = may be deleted
  VARIANT 10..11: note = may be deleted
  VARIANT 11: note = may be deleted
  VARIANT 7..11: note = may be deleted
  VARIANT 7: note = L, I, or V
GYRGISXXXXX

SEQ ID NO: 222 - protein, 11 aa, synthetic construct
  VARIANT 8: note = A, G, or V
  VARIANT 9: note = K, N, or Q
  VARIANT 10: note = W or F
  VARIANT 11: note = M, M-NH2, L, I, V, A, or G
  VARIANT 8..11: note = may be deleted
  VARIANT 9..11: note = may be deleted
  VARIANT 10..11: note = may be deleted
  VARIANT 11: note = may be deleted
  VARIANT 7..11: note = may be deleted
  VARIANT 7: note = L, I, or V
GYRGYTXXXXX

SEQ ID NO: 223 - protein, 11 aa, synthetic construct
  VARIANT 8: note = A, G, or V
  VARIANT 9: note = K, N, or Q
  VARIANT 10: note = W or F
  VARIANT 11: note = M, M-NH2, L, I, V, A, or G
  VARIANT 8..11: note = may be deleted
  VARIANT 9..11: note = may be deleted
  VARIANT 10..11: note = may be deleted
  VARIANT 11: note = may be deleted
  VARIANT 7..11: note = may be deleted
  VARIANT 7: note = L, I, or V
GYRGITXXXXX

SEQ ID NO: 224 - protein, 11 aa, synthetic construct
  VARIANT 8: note = A, G, or V
  VARIANT 9: note = K, N, or Q
  VARIANT 10: note = W or F
  VARIANT 11: note = M, M-NH2, L, I, V, A, or G
  VARIANT 8..11: note = may be deleted
  VARIANT 9..11: note = may be deleted
  VARIANT 10..11: note = may be deleted
  VARIANT 11: note = may be deleted
  VARIANT 7..11: note = may be deleted
  VARIANT 7: note = L, I, or V
  VARIANT 6: note = S or T
GYKGIXXXXXX

SEQ ID NO: 225 - protein, 11 aa, synthetic construct
  VARIANT 8: note = A, G, or V
  VARIANT 9: note = K, N, or Q
  VARIANT 10: note = W or F
  VARIANT 11: note = M, M-NH2, L, I, V, A, or G
  VARIANT 8..11: note = may be deleted
  VARIANT 9..11: note = may be deleted
  VARIANT 10..11: note = may be deleted
  VARIANT 11: note = may be deleted
  VARIANT 7..11: note = may be deleted
  VARIANT 7: note = L, I, or V
  VARIANT 6: note = S or T
GYKGYXXXXXX

SEQ ID NO: 226 - protein, 11 aa, synthetic construct
  VARIANT 8: note = A, G, or V
  VARIANT 9: note = K, N, or Q
  VARIANT 10: note = W or F
  VARIANT 11: note = M, M-NH2, L, I, V, A, or G
  VARIANT 8..11: note = may be deleted
  VARIANT 9..11: note = may be deleted
  VARIANT 10..11: note = may be deleted
  VARIANT 11: note = may be deleted
  VARIANT 7..11: note = may be deleted
  VARIANT 7: note = L, I, or V
  VARIANT 5: note = I, Y, Q, N, L, or F
GYKGXSXXXXX

SEQ ID NO: 227 - protein, 11 aa, synthetic construct
  VARIANT 8: note = A, G, or V
  VARIANT 9: note = K, N, or Q
  VARIANT 10: note = W or F
  VARIANT 11: note = M, M-NH2, L, I, V, A, or G
  VARIANT 8..11: note = may be deleted
  VARIANT 9..11: note = may be deleted
  VARIANT 10..11: note = may be deleted
  VARIANT 11: note = may be deleted
  VARIANT 7..11: note = may be deleted
  VARIANT 7: note = L, I, or V
  VARIANT 5: note = I, Y, Q, N, L, or F
GYKGXTXXXXX

SEQ ID NO: 228 - protein, 11 aa, synthetic construct
  VARIANT 8: note = A, G, or V
  VARIANT 9: note = K, N, or Q
  VARIANT 10: note = W or F
  VARIANT 11: note = M, M-NH2, L, I, V, A, or G
  VARIANT 8..11: note = may be deleted
  VARIANT 9..11: note = may be deleted
  VARIANT 10..11: note = may be deleted
  VARIANT 11: note = may be deleted
  VARIANT 7..11: note = may be deleted
  VARIANT 7: note = L, I, or V
  VARIANT 4: note = G or A
GYKXISXXXXX

SEQ ID NO: 229 - protein, 11 aa, synthetic construct
  VARIANT 8: note = A, G, or V
  VARIANT 9: note = K, N, or Q
  VARIANT 10: note = W or F
  VARIANT 11: note = M, M-NH2, L, I, V, A, or G
  VARIANT 8..11: note = may be deleted
  VARIANT 9..11: note = may be deleted
  VARIANT 10..11: note = may be deleted
  VARIANT 11: note = may be deleted
  VARIANT 7..11: note = may be deleted
  VARIANT 7: note = L, I, or V
  VARIANT 4: note = G or A
GYKXITXXXXX

SEQ ID NO: 230 - protein, 11 aa, synthetic construct
  VARIANT 8: note = A, G, or V
  VARIANT 9: note = K, N, or Q
  VARIANT 10: note = W or F
  VARIANT 11: note = M, M-NH2, L, I, V, A, or G
  VARIANT 8..11: note = may be deleted
  VARIANT 9..11: note = may be deleted
  VARIANT 10..11: note = may be deleted
  VARIANT 11: note = may be deleted
  VARIANT 7..11: note = may be deleted
  VARIANT 7: note = L, I, or V
  VARIANT 4: note = G or A
GYKXYSXXXXX

SEQ ID NO: 231 - protein, 11 aa, synthetic construct
  VARIANT 8: note = A, G, or V
  VARIANT 9: note = K, N, or Q
  VARIANT 10: note = W or F
  VARIANT 11: note = M, M-NH2, L, I, V, A, or G
  VARIANT 8..11: note = may be deleted
  VARIANT 9..11: note = may be deleted
  VARIANT 10..11: note = may be deleted
  VARIANT 11: note = may be deleted
  VARIANT 7..11: note = may be deleted
  VARIANT 7: note = L, I, or V
  VARIANT 4: note = G or A
GYKXYTXXXXX

SEQ ID NO: 232 - protein, 11 aa, synthetic construct
  VARIANT 8: note = A, G, or V
  VARIANT 9: note = K, N, or Q
  VARIANT 10: note = W or F
  VARIANT 11: note = M, M-NH2, L, I, V, A, or G
  VARIANT 8..11: note = may be deleted
  VARIANT 9..11: note = may be deleted
  VARIANT 10..11: note = may be deleted
  VARIANT 11: note = may be deleted
  VARIANT 7..11: note = may be deleted
  VARIANT 7: note = L, I, or V
GYKGYSXXXXX

SEQ ID NO: 233 - protein, 11 aa, synthetic construct
  VARIANT 8: note = A, G, or V
  VARIANT 9: note = K, N, or Q
  VARIANT 10: note = W or F
  VARIANT 11: note = M, M-NH2, L, I, V, A, or G
  VARIANT 8..11: note = may be deleted
  VARIANT 9..11: note = may be deleted
  VARIANT 10..11: note = may be deleted
  VARIANT 11: note = may be deleted
  VARIANT 7..11: note = may be deleted
  VARIANT 7: note = L, I, or V
GYKGISXXXXX

SEQ ID NO: 234 - protein, 11 aa, synthetic construct
  VARIANT 8: note = A, G, or V
  VARIANT 9: note = K, N, or Q
  VARIANT 10: note = W or F
  VARIANT 11: note = M, M-NH2, L, I, V, A, or G
  VARIANT 8..11: note = may be deleted
  VARIANT 9..11: note = may be deleted
  VARIANT 10..11: note = may be deleted
  VARIANT 11: note = may be deleted
  VARIANT 7..11: note = may be deleted
  VARIANT 7: note = L, I, or V
GYKGYTXXXXX

SEQ ID NO: 235 - protein, 11 aa, synthetic construct
  VARIANT 8: note = A, G, or V
  VARIANT 9: note = K, N, or Q
  VARIANT 10: note = W or F
  VARIANT 11: note = M, M-NH2, L, I, V, A, or G
  VARIANT 8..11: note = may be deleted
  VARIANT 9..11: note = may be deleted
  VARIANT 10..11: note = may be deleted
  VARIANT 11: note = may be deleted
  VARIANT 7..11: note = may be deleted
  VARIANT 7: note = L, I, or V
GYKGITXXXXX

SEQ ID NO: 236 - protein, 11 aa, synthetic construct
  VARIANT 8: note = A, G, or V
  VARIANT 9: note = K, N, or Q
  VARIANT 10: note = W or F
  VARIANT 11: note = M, M-NH2, L, I, V, A, or G
  VARIANT 8..11: note = may be deleted
  VARIANT 9..11: note = may be deleted
  VARIANT 10..11: note = may be deleted
  VARIANT 11: note = may be deleted
  VARIANT 7..11: note = may be deleted
  VARIANT 7: note = L, I, or V
  VARIANT 6: note = S or T
GYLGIXXXXXX

SEQ ID NO: 237 - protein, 11 aa, synthetic construct
  VARIANT 8: note = A, G, or V
  VARIANT 9: note = K, N, or Q
  VARIANT 10: note = W or F
  VARIANT 11: note = M, M-NH2, L, I, V, A, or G
  VARIANT 8..11: note = may be deleted
  VARIANT 9..11: note = may be deleted
  VARIANT 10..11: note = may be deleted
  VARIANT 11: note = may be deleted
  VARIANT 7..11: note = may be deleted
  VARIANT 7: note = L, I, or V
  VARIANT 6: note = S or T
GYLGYXXXXXX

SEQ ID NO: 238 - protein, 11 aa, synthetic construct
  VARIANT 8: note = A, G, or V
  VARIANT 9: note = K, N, or Q
  VARIANT 10: note = W or F
  VARIANT 11: note = M, M-NH2, L, I, V, A, or G
  VARIANT 8..11: note = may be deleted
  VARIANT 9..11: note = may be deleted
  VARIANT 10..11: note = may be deleted
  VARIANT 11: note = may be deleted
  VARIANT 7..11: note = may be deleted
  VARIANT 7: note = L, I, or V
  VARIANT 5: note = I, Y, Q, N, L, or F
GYLGXSXXXXX

SEQ ID NO: 239 - protein, 11 aa, synthetic construct
  VARIANT 8: note = A, G, or V
  VARIANT 9: note = K, N, or Q
  VARIANT 10: note = W or F
  VARIANT 11: note = M, M-NH2, L, I, V, A, or G
  VARIANT 8..11: note = may be deleted
  VARIANT 9..11: note = may be deleted
  VARIANT 10..11: note = may be deleted
  VARIANT 11: note = may be deleted
  VARIANT 7..11: note = may be deleted
  VARIANT 7: note = L, I, or V
  VARIANT 5: note = I, Y, Q, N, L, or F
GYLGXTXXXXX

SEQ ID NO: 240 - protein, 11 aa, synthetic construct
  VARIANT 8: note = A, G, or V
  VARIANT 9: note = K, N, or Q
  VARIANT 10: note = W or F
  VARIANT 11: note = M, M-NH2, L, I, V, A, or G
  VARIANT 8..11: note = may be deleted
  VARIANT 9..11: note = may be deleted
  VARIANT 10..11: note = may be deleted
  VARIANT 11: note = may be deleted
  VARIANT 7..11: note = may be deleted
  VARIANT 7: note = L, I, or V
  VARIANT 4: note = G or A
GYLXISXXXXX

SEQ ID NO: 241 - protein, 11 aa, synthetic construct
  VARIANT 8: note = A, G, or V
  VARIANT 9: note = K, N, or Q
  VARIANT 10: note = W or F
  VARIANT 11: note = M, M-NH2, L, I, V, A, or G
  VARIANT 8..11: note = may be deleted
  VARIANT 9..11: note = may be deleted
  VARIANT 10..11: note = may be deleted
  VARIANT 11: note = may be deleted
  VARIANT 7..11: note = may be deleted
  VARIANT 7: note = L, I, or V
  VARIANT 4: note = G or A
GYLXITXXXXX

SEQ ID NO: 242 - protein, 11 aa, synthetic construct
  VARIANT 8: note = A, G, or V
  VARIANT 9: note = K, N, or Q
  VARIANT 10: note = W or F
  VARIANT 11: note = M, M-NH2, L, I, V, A, or G
  VARIANT 8..11: note = may be deleted
  VARIANT 9..11: note = may be deleted
  VARIANT 10..11: note = may be deleted
  VARIANT 11: note = may be deleted
  VARIANT 7..11: note = may be deleted
  VARIANT 7: note = L, I, or V
  VARIANT 4: note = G or A
GYLXYSXXXXX

SEQ ID NO: 243 - protein, 11 aa, synthetic construct
  VARIANT 8: note = A, G, or V
  VARIANT 9: note = K, N, or Q
  VARIANT 10: note = W or F
  VARIANT 11: note = M, M-NH2, L, I, V, A, or G
  VARIANT 8..11: note = may be deleted
  VARIANT 9..11: note = may be deleted
  VARIANT 10..11: note = may be deleted
  VARIANT 11: note = may be deleted
  VARIANT 7..11: note = may be deleted
  VARIANT 7: note = L, I, or V
  VARIANT 4: note = G or A
GYLXYTXXXXX

SEQ ID NO: 244 - protein, 11 aa, synthetic construct
  VARIANT 8: note = A, G, or V
  VARIANT 9: note = K, N, or Q
  VARIANT 10: note = W or F
  VARIANT 11: note = M, M-NH2, L, I, V, A, or G
  VARIANT 8..11: note = may be deleted
  VARIANT 9..11: note = may be deleted
  VARIANT 10..11: note = may be deleted
  VARIANT 11: note = may be deleted
  VARIANT 7..11: note = may be deleted
  VARIANT 7: note = L, I, or V
GYLGYSXXXXX

SEQ ID NO: 245 - protein, 11 aa, synthetic construct
  VARIANT 8: note = A, G, or V
  VARIANT 9: note = K, N, or Q
  VARIANT 10: note = W or F
  VARIANT 11: note = M, M-NH2, L, I, V, A, or G
  VARIANT 8..11: note = may be deleted
  VARIANT 9..11: note = may be deleted
  VARIANT 10..11: note = may be deleted
  VARIANT 11: note = may be deleted
  VARIANT 7..11: note = may be deleted
  VARIANT 7: note = L, I, or V
GYLGISXXXXX

SEQ ID NO: 246 - protein, 11 aa, synthetic construct
  VARIANT 8: note = A, G, or V
  VARIANT 9: note = K, N, or Q
  VARIANT 10: note = W or F
  VARIANT 11: note = M, M-NH2, L, I, V, A, or G
  VARIANT 8..11: note = may be deleted
  VARIANT 9..11: note = may be deleted
  VARIANT 10..11: note = may be deleted
  VARIANT 11: note = may be deleted
  VARIANT 7..11: note = may be deleted
  VARIANT 7: note = L, I, or V
GYLGYTXXXXX

SEQ ID NO: 247 - protein, 11 aa, synthetic construct
  VARIANT 8: note = A, G, or V
  VARIANT 9: note = K, N, or Q
  VARIANT 10: note = W or F
  VARIANT 11: note = M, M-NH2, L, I, V, A, or G
  VARIANT 8..11: note = may be deleted
  VARIANT 9..11: note = may be deleted
  VARIANT 10..11: note = may be deleted
  VARIANT 11: note = may be deleted
  VARIANT 7..11: note = may be deleted
  VARIANT 7: note = L, I, or V
GYLGITXXXXX

SEQ ID NO: 248 - protein, 11 aa, synthetic construct
  VARIANT 8: note = A, G, or V
  VARIANT 9: note = K, N, or Q
  VARIANT 10: note = W or F
  VARIANT 11: note = M, M-NH2, L, I, V, A, or G
  VARIANT 8..11: note = may be deleted
  VARIANT 9..11: note = may be deleted
  VARIANT 10..11: note = may be deleted
  VARIANT 11: note = may be deleted
  VARIANT 7..11: note = may be deleted
  VARIANT 7: note = L, I, or V
  VARIANT 6: note = S or T
GFRGIXXXXXX

SEQ ID NO: 249 - protein, 11 aa, synthetic construct
  VARIANT 8: note = A, G, or V
  VARIANT 9: note = K, N, or Q
  VARIANT 10: note = W or F
  VARIANT 11: note = M, M-NH2, L, I, V, A, or G
  VARIANT 8..11: note = may be deleted
  VARIANT 9..11: note = may be deleted
  VARIANT 10..11: note = may be deleted
  VARIANT 11: note = may be deleted
  VARIANT 7..11: note = may be deleted
  VARIANT 7: note = L, I, or V
  VARIANT 6: note = S or T
GFRGYXXXXXX

SEQ ID NO: 250 - protein, 11 aa, synthetic construct
  VARIANT 8: note = A, G, or V
  VARIANT 9: note = K, N, or Q
  VARIANT 10: note = W or F
  VARIANT 11: note = M, M-NH2, L, I, V, A, or G
  VARIANT 8..11: note = may be deleted
  VARIANT 9..11: note = may be deleted
  VARIANT 10..11: note = may be deleted
  VARIANT 11: note = may be deleted
  VARIANT 7..11: note = may be deleted
  VARIANT 7: note = L, I, or V
  VARIANT 5: note = I, Y, Q, N, L, or F
GFRGXSXXXXX

SEQ ID NO: 251 - protein, 11 aa, synthetic construct
  VARIANT 8: note = A, G, or V
  VARIANT 9: note = K, N, or Q
  VARIANT 10: note = W or F
  VARIANT 11: note = M, M-NH2, L, I, V, A, or G
  VARIANT 8..11: note = may be deleted
  VARIANT 9..11: note = may be deleted
  VARIANT 10..11: note = may be deleted
  VARIANT 11: note = may be deleted
  VARIANT 7..11: note = may be deleted
  VARIANT 7: note = L, I, or V
  VARIANT 5: note = I, Y, Q, N, L, or F
GFRGXTXXXXX

SEQ ID NO: 252 - protein, 11 aa, synthetic construct
  VARIANT 8: note = A, G, or V
  VARIANT 9: note = K, N, or Q
  VARIANT 10: note = W or F
  VARIANT 11: note = M, M-NH2, L, I, V, A, or G
  VARIANT 8..11: note = may be deleted
  VARIANT 9..11: note = may be deleted
  VARIANT 10..11: note = may be deleted
  VARIANT 11: note = may be deleted
  VARIANT 7..11: note = may be deleted
  VARIANT 7: note = L, I, or V
  VARIANT 4: note = G or A
GFRXISXXXXX

SEQ ID NO: 253 - protein, 11 aa, synthetic construct
  VARIANT 8: note = A, G, or V
  VARIANT 9: note = K, N, or Q
  VARIANT 10: note = W or F
  VARIANT 11: note = M, M-NH2, L, I, V, A, or G
  VARIANT 8..11: note = may be deleted
  VARIANT 9..11: note = may be deleted
  VARIANT 10..11: note = may be deleted
  VARIANT 11: note = may be deleted
  VARIANT 7..11: note = may be deleted
  VARIANT 7: note = L, I, or V
  VARIANT 4: note = G or A
GFRXITXXXXX

SEQ ID NO: 254 - protein, 11 aa, synthetic construct
  VARIANT 8: note = A, G, or V
  VARIANT 9: note = K, N, or Q
  VARIANT 10: note = W or F
  VARIANT 11: note = M, M-NH2, L, I, V, A, or G
  VARIANT 8..11: note = may be deleted
  VARIANT 9..11: note = may be deleted
  VARIANT 10..11: note = may be deleted
  VARIANT 11: note = may be deleted
  VARIANT 7..11: note = may be deleted
  VARIANT 7: note = L, I, or V
  VARIANT 4: note = G or A
GFRXYSXXXXX

SEQ ID NO: 255 - protein, 11 aa, synthetic construct
  VARIANT 8: note = A, G, or V
  VARIANT 9: note = K, N, or Q
  VARIANT 10: note = W or F
  VARIANT 11: note = M, M-NH2, L, I, V, A, or G
  VARIANT 8..11: note = may be deleted
  VARIANT 9..11: note = may be deleted
  VARIANT 10..11: note = may be deleted
  VARIANT 11: note = may be deleted
  VARIANT 7..11: note = may be deleted
  VARIANT 7: note = L, I, or V
  VARIANT 4: note = G or A
GFRXYTXXXXX

SEQ ID NO: 256 - protein, 11 aa, synthetic construct
  VARIANT 8: note = A, G, or V
  VARIANT 9: note = K, N, or Q
  VARIANT 10: note = W or F
  VARIANT 11: note = M, M-NH2, L, I, V, A, or G
  VARIANT 8..11: note = may be deleted
  VARIANT 9..11: note = may be deleted
  VARIANT 10..11: note = may be deleted
  VARIANT 11: note = may be deleted
  VARIANT 7..11: note = may be deleted
  VARIANT 7: note = L, I, or V
GFRGYSXXXXX

SEQ ID NO: 257 - protein, 11 aa, synthetic construct
  VARIANT 8: note = A, G, or V
  VARIANT 9: note = K, N, or Q
  VARIANT 10: note = W or F
  VARIANT 11: note = M, M-NH2, L, I, V, A, or G
  VARIANT 8..11: note = may be deleted
  VARIANT 9..11: note = may be deleted
  VARIANT 10..11: note = may be deleted
  VARIANT 11: note = may be deleted
  VARIANT 7..11: note = may be deleted
  VARIANT 7: note = L, I, or V
GFRGISXXXXX

SEQ ID NO: 258 - protein, 11 aa, synthetic construct
  VARIANT 8: note = A, G, or V
  VARIANT 9: note = K, N, or Q
  VARIANT 10: note = W or F
  VARIANT 11: note = M, M-NH2, L, I, V, A, or G
  VARIANT 8..11: note = may be deleted
  VARIANT 9..11: note = may be deleted
  VARIANT 10..11: note = may be deleted
  VARIANT 11: note = may be deleted
  VARIANT 7..11: note = may be deleted
  VARIANT 7: note = L, I, or V
GFRGYTXXXXX

SEQ ID NO: 259 - protein, 11 aa, synthetic construct
  VARIANT 8: note = A, G, or V
  VARIANT 9: note = K, N, or Q
  VARIANT 10: note = W or F
  VARIANT 11: note = M, M-NH2, L, I, V, A, or G
  VARIANT 8..11: note = may be deleted
  VARIANT 9..11: note = may be deleted
  VARIANT 10..11: note = may be deleted
  VARIANT 11: note = may be deleted
  VARIANT 7..11: note = may be deleted
  VARIANT 7: note = L, I, or V
GFRGITXXXXX

SEQ ID NO: 260 - protein, 11 aa, synthetic construct
  VARIANT 8: note = A, G, or V
  VARIANT 9: note = K, N, or Q
  VARIANT 10: note = W or F
  VARIANT 11: note = M, M-NH2, L, I, V, A, or G
  VARIANT 8..11: note = may be deleted
  VARIANT 9..11: note = may be deleted
  VARIANT 10..11: note = may be deleted
  VARIANT 11: note = may be deleted
  VARIANT 7..11: note = may be deleted
  VARIANT 7: note = L, I, or V
  VARIANT 6: note = S or T
GFKGIXXXXXX

SEQ ID NO: 261 - protein, 11 aa, synthetic construct
  VARIANT 8: note = A, G, or V
  VARIANT 9: note = K, N, or Q
  VARIANT 10: note = W or F
  VARIANT 11: note = M, M-NH2, L, I, V, A, or G
  VARIANT 8..11: note = may be deleted
  VARIANT 9..11: note = may be deleted
  VARIANT 10..11: note = may be deleted
  VARIANT 11: note = may be deleted
  VARIANT 7..11: note = may be deleted
  VARIANT 7: note = L, I, or V
  VARIANT 6: note = S or T
GFKGYXXXXXX

SEQ ID NO: 262 - protein, 11 aa, synthetic construct
  VARIANT 8: note = A, G, or V
  VARIANT 9: note = K, N, or Q
  VARIANT 10: note = W or F
  VARIANT 11: note = M, M-NH2, L, I, V, A, or G
  VARIANT 8..11: note = may be deleted
  VARIANT 9..11: note = may be deleted
  VARIANT 10..11: note = may be deleted
  VARIANT 11: note = may be deleted
  VARIANT 7..11: note = may be deleted
  VARIANT 7: note = L, I, or V
  VARIANT 5: note = I, Y, Q, N, L, or F
GFKGXSXXXXX

SEQ ID NO: 263 - protein, 11 aa, synthetic construct
  VARIANT 8: note = A, G, or V
  VARIANT 9: note = K, N, or Q
  VARIANT 10: note = W or F
  VARIANT 11: note = M, M-NH2, L, I, V, A, or G
  VARIANT 8..11: note = may be deleted
  VARIANT 9..11: note = may be deleted
  VARIANT 10..11: note = may be deleted
  VARIANT 11: note = may be deleted
  VARIANT 7..11: note = may be deleted
  VARIANT 7: note = L, I, or V
  VARIANT 5: note = I, Y, Q, N, L, or F
GFKGXTXXXXX

SEQ ID NO: 264 - protein, 11 aa, synthetic construct
  VARIANT 8: note = A, G, or V
  VARIANT 9: note = K, N, or Q
  VARIANT 10: note = W or F
  VARIANT 11: note = M, M-NH2, L, I, V, A, or G
  VARIANT 8..11: note = may be deleted
  VARIANT 9..11: note = may be deleted
  VARIANT 10..11: note = may be deleted
  VARIANT 11: note = may be deleted
  VARIANT 7..11: note = may be deleted
  VARIANT 7: note = L, I, or V
  VARIANT 4: note = G or A
GFKXISXXXXX

SEQ ID NO: 265 - protein, 11 aa, synthetic construct
  VARIANT 8: note = A, G, or V
  VARIANT 9: note = K, N, or Q
  VARIANT 10: note = W or F
  VARIANT 11: note = M, M-NH2, L, I, V, A, or G
  VARIANT 8..11: note = may be deleted
  VARIANT 9..11: note = may be deleted
  VARIANT 10..11: note = may be deleted
  VARIANT 11: note = may be deleted
  VARIANT 7..11: note = may be deleted
  VARIANT 7: note = L, I, or V
  VARIANT 4: note = G or A
GFKXITXXXXX

SEQ ID NO: 266 - protein, 11 aa, synthetic construct
  VARIANT 8: note = A, G, or V
  VARIANT 9: note = K, N, or Q
  VARIANT 10: note = W or F
  VARIANT 11: note = M, M-NH2, L, I, V, A, or G
  VARIANT 8..11: note = may be deleted
  VARIANT 9..11: note = may be deleted
  VARIANT 10..11: note = may be deleted
  VARIANT 11: note = may be deleted
  VARIANT 7..11: note = may be deleted
  VARIANT 7: note = L, I, or V
  VARIANT 4: note = G or A
GFKXYSXXXXX

SEQ ID NO: 267 - protein, 11 aa, synthetic construct
  VARIANT 8: note = A, G, or V
  VARIANT 9: note = K, N, or Q
  VARIANT 10: note = W or F
  VARIANT 11: note = M, M-NH2, L, I, V, A, or G
  VARIANT 8..11: note = may be deleted
  VARIANT 9..11: note = may be deleted
  VARIANT 10..11: note = may be deleted
  VARIANT 11: note = may be deleted
  VARIANT 7..11: note = may be deleted
  VARIANT 7: note = L, I, or V
  VARIANT 4: note = G or A
GFKXYTXXXXX

SEQ ID NO: 268 - protein, 11 aa, synthetic construct
  VARIANT 8: note = A, G, or V
  VARIANT 9: note = K, N, or Q
  VARIANT 10: note = W or F
  VARIANT 11: note = M, M-NH2, L, I, V, A, or G
  VARIANT 8..11: note = may be deleted
  VARIANT 9..11: note = may be deleted
  VARIANT 10..11: note = may be deleted
  VARIANT 11: note = may be deleted
  VARIANT 7..11: note = may be deleted
  VARIANT 7: note = L, I, or V
GFKGYSXXXXX

SEQ ID NO: 269 - protein, 11 aa, synthetic construct
  VARIANT 8: note = A, G, or V
  VARIANT 9: note = K, N, or Q
  VARIANT 10: note = W or F
  VARIANT 11: note = M, M-NH2, L, I, V, A, or G
  VARIANT 8..11: note = may be deleted
  VARIANT 9..11: note = may be deleted
  VARIANT 10..11: note = may be deleted
  VARIANT 11: note = may be deleted
  VARIANT 7..11: note = may be deleted
  VARIANT 7: note = L, I, or V
GFKGISXXXXX

SEQ ID NO: 270 - protein, 11 aa, synthetic construct
  VARIANT 8: note = A, G, or V
  VARIANT 9: note = K, N, or Q
  VARIANT 10: note = W or F
  VARIANT 11: note = M, M-NH2, L, I, V, A, or G
  VARIANT 8..11: note = may be deleted
  VARIANT 9..11: note = may be deleted
  VARIANT 10..11: note = may be deleted
  VARIANT 11: note = may be deleted
  VARIANT 7..11: note = may be deleted
  VARIANT 7: note = L, I, or V
GFKGYTXXXXX

SEQ ID NO: 271 - protein, 11 aa, synthetic construct
  VARIANT 8: note = A, G, or V
  VARIANT 9: note = K, N, or Q
  VARIANT 10: note = W or F
  VARIANT 11: note = M, M-NH2, L, I, V, A, or G
  VARIANT 8..11: note = may be deleted
  VARIANT 9..11: note = may be deleted
  VARIANT 10..11: note = may be deleted
  VARIANT 11: note = may be deleted
  VARIANT 7..11: note = may be deleted
  VARIANT 7: note = L, I, or V
GFKGITXXXXX

SEQ ID NO: 272 - protein, 11 aa, synthetic construct
  VARIANT 8: note = A, G, or V
  VARIANT 9: note = K, N, or Q
  VARIANT 10: note = W or F
  VARIANT 11: note = M, M-NH2, L, I, V, A, or G
  VARIANT 8..11: note = may be deleted
  VARIANT 9..11: note = may be deleted
  VARIANT 10..11: note = may be deleted
  VARIANT 11: note = may be deleted
  VARIANT 7..11: note = may be deleted
  VARIANT 7: note = L, I, or V
  VARIANT 6: note = S or T
GFLGIXXXXXX

SEQ ID NO: 273 - protein, 11 aa, synthetic construct
  VARIANT 8: note = A, G, or V
  VARIANT 9: note = K, N, or Q
  VARIANT 10: note = W or F
  VARIANT 11: note = M, M-NH2, L, I, V, A, or G
  VARIANT 8..11: note = may be deleted
  VARIANT 9..11: note = may be deleted
  VARIANT 10..11: note = may be deleted
  VARIANT 11: note = may be deleted
  VARIANT 7..11: note = may be deleted
  VARIANT 7: note = L, I, or V
  VARIANT 6: note = S or T
GFLGYXXXXXX

SEQ ID NO: 274 - protein, 11 aa, synthetic construct
  VARIANT 8: note = A, G, or V
  VARIANT 9: note = K, N, or Q
  VARIANT 10: note = W or F
  VARIANT 11: note = M, M-NH2, L, I, V, A, or G
  VARIANT 8..11: note = may be deleted
  VARIANT 9..11: note = may be deleted
  VARIANT 10..11: note = may be deleted
  VARIANT 11: note = may be deleted
  VARIANT 7..11: note = may be deleted
  VARIANT 7: note = L, I, or V
  VARIANT 5: note = I, Y, Q, N, L, or F
GYLGXSXXXXX

SEQ ID NO: 275 - protein, 11 aa, synthetic construct
  VARIANT 8: note = A, G, or V
  VARIANT 9: note = K, N, or Q
  VARIANT 10: note = W or F
  VARIANT 11: note = M, M-NH2, L, I, V, A, or G
  VARIANT 8..11: note = may be deleted
  VARIANT 9..11: note = may be deleted
  VARIANT 10..11: note = may be deleted
  VARIANT 11: note = may be deleted
  VARIANT 7..11: note = may be deleted
  VARIANT 7: note = L, I, or V
  VARIANT 5: note = I, Y, Q, N, L, or F
GFLGXTXXXXX

SEQ ID NO: 276 - protein, 11 aa, synthetic construct
  VARIANT 8: note = A, G, or V
  VARIANT 9: note = K, N, or Q
  VARIANT 10: note = W or F
  VARIANT 11: note = M, M-NH2, L, I, V, A, or G
  VARIANT 8..11: note = may be deleted
  VARIANT 9..11: note = may be deleted
  VARIANT 10..11: note = may be deleted
  VARIANT 11: note = may be deleted
  VARIANT 7..11: note = may be deleted
  VARIANT 7: note = L, I, or V
  VARIANT 4: note = G or A
GFLXISXXXXX

SEQ ID NO: 277 - protein, 11 aa, synthetic construct
  VARIANT 8: note = A, G, or V
  VARIANT 9: note = K, N, or Q
  VARIANT 10: note = W or F
  VARIANT 11: note = M, M-NH2, L, I, V, A, or G
  VARIANT 8..11: note = may be deleted
  VARIANT 9..11: note = may be deleted
  VARIANT 10..11: note = may be deleted
  VARIANT 11: note = may be deleted
  VARIANT 7..11: note = may be deleted
  VARIANT 7: note = L, I, or V
  VARIANT 4: note = G or A
GFLXITXXXXX

SEQ ID NO: 278 - protein, 11 aa, synthetic construct
  VARIANT 8: note = A, G, or V
  VARIANT 9: note = K, N, or Q
  VARIANT 10: note = W or F
  VARIANT 11: note = M, M-NH2, L, I, V, A, or G
  VARIANT 8..11: note = may be deleted
  VARIANT 9..11: note = may be deleted
  VARIANT 10..11: note = may be deleted
  VARIANT 11: note = may be deleted
  VARIANT 7..11: note = may be deleted
  VARIANT 7: note = L, I, or V
  VARIANT 4: note = G or A
GFLXYSXXXXX

SEQ ID NO: 279 - protein, 11 aa, synthetic construct
  VARIANT 8: note = A, G, or V
  VARIANT 9: note = K, N, or Q
  VARIANT 10: note = W or F
  VARIANT 11: note = M, M-NH2, L, I, V, A, or G
  VARIANT 8..11: note = may be deleted
  VARIANT 9..11: note = may be deleted
  VARIANT 10..11: note = may be deleted
  VARIANT 11: note = may be deleted
  VARIANT 7..11: note = may be deleted
  VARIANT 7: note = L, I, or V
  VARIANT 4: note = G or A
GFLXYTXXXXX

SEQ ID NO: 280 - protein, 11 aa, synthetic construct
  VARIANT 8: note = A, G, or V
  VARIANT 9: note = K, N, or Q
  VARIANT 10: note = W or F
  VARIANT 11: note = M, M-NH2, L, I, V, A, or G
  VARIANT 8..11: note = may be deleted
  VARIANT 9..11: note = may be deleted
  VARIANT 10..11: note = may be deleted
  VARIANT 11: note = may be deleted
  VARIANT 7..11: note = may be deleted
  VARIANT 7: note = L, I, or V
GFLGYSXXXXX

SEQ ID NO: 281 - protein, 11 aa, synthetic construct
  VARIANT 8: note = A, G, or V
  VARIANT 9: note = K, N, or Q
  VARIANT 10: note = W or F
  VARIANT 11: note = M, M-NH2, L, I, V, A, or G
  VARIANT 8..11: note = may be deleted
  VARIANT 9..11: note = may be deleted
  VARIANT 10..11: note = may be deleted
  VARIANT 11: note = may be deleted
  VARIANT 7..11: note = may be deleted
  VARIANT 7: note = L, I, or V
GFLGISXXXXX

SEQ ID NO: 282 - protein, 11 aa, synthetic construct
  VARIANT 8: note = A, G, or V
  VARIANT 9: note = K, N, or Q
  VARIANT 10: note = W or F
  VARIANT 11: note = M, M-NH2, L, I, V, A, or G
  VARIANT 8..11: note = may be deleted
  VARIANT 9..11: note = may be deleted
  VARIANT 10..11: note = may be deleted
  VARIANT 11: note = may be deleted
  VARIANT 7..11: note = may be deleted
  VARIANT 7: note = L, I, or V
GFLGYTXXXXX

SEQ ID NO: 283 - protein, 11 aa, synthetic construct
  VARIANT 8: note = A, G, or V
  VARIANT 9: note = K, N, or Q
  VARIANT 10: note = W or F
  VARIANT 11: note = M, M-NH2, L, I, V, A, or G
  VARIANT 8..11: note = may be deleted
  VARIANT 9..11: note = may be deleted
  VARIANT 10..11: note = may be deleted
  VARIANT 11: note = may be deleted
  VARIANT 7..11: note = may be deleted
  VARIANT 7: note = L, I, or V
GFLGITXXXXX

SEQ ID NO: 284 - protein, 11 aa, synthetic construct
  VARIANT 1: note = G or A
  VARIANT 2: note = Y, F, or W
  VARIANT 9: note = K, N, or Q
  VARIANT 10: note = W or F
  VARIANT 11: note = M, M-NH2, L, I, V, A, or G
  VARIANT 1..2: note = may be deleted
  VARIANT 1: note = may be deleted
  VARIANT 9..11: note = may be deleted
  VARIANT 10..11: note = may be deleted
  VARIANT 11: note = may be deleted
  VARIANT 6: note = S or T
  VARIANT 8..11: note = may be deleted
  VARIANT 8: note = A, G or V
XXRGIXLXXXX

SEQ ID NO: 285 - protein, 11 aa, synthetic construct
  VARIANT 1: note = G or A
  VARIANT 2: note = Y, F, or W
  VARIANT 9: note = K, N, or Q
  VARIANT 10: note = W or F
  VARIANT 11: note = M, M-NH2, L, I, V, A, or G
  VARIANT 1..2: note = may be deleted
  VARIANT 1: note = may be deleted
  VARIANT 9..11: note = may be deleted
  VARIANT 10..11: note = may be deleted
  VARIANT 11: note = may be deleted
  VARIANT 6: note = S or T
  VARIANT 8..11: note = may be deleted
  VARIANT 8: note = A, G or V
XXRGYXLXXXX

SEQ ID NO: 286 - protein, 11 aa, synthetic construct
  VARIANT 1: note = G or A
  VARIANT 2: note = Y, F, or W
  VARIANT 9: note = K, N, or Q
  VARIANT 10: note = W or F
  VARIANT 11: note = M, M-NH2, L, I, V, A, or G
  VARIANT 1..2: note = may be deleted
  VARIANT 1: note = may be deleted
  VARIANT 9..11: note = may be deleted
  VARIANT 10..11: note = may be deleted
  VARIANT 11: note = may be deleted
  VARIANT 5: note = I, Y, Q, N, L, or F
  VARIANT 8..11: note = may be deleted
  VARIANT 8: note = A, G or V
XXRGXSLXXXX

SEQ ID NO: 287 - protein, 11 aa, synthetic construct
  VARIANT 1: note = G or A
  VARIANT 2: note = Y, F, or W
  VARIANT 9: note = K, N, or Q
  VARIANT 10: note = W or F
  VARIANT 11: note = M, M-NH2, L, I, V, A, or G
  VARIANT 1..2: note = may be deleted
  VARIANT 1: note = may be deleted
  VARIANT 9..11: note = may be deleted
  VARIANT 10..11: note = may be deleted
  VARIANT 11: note = may be deleted
  VARIANT 5: note = I, Y, Q, N, L, or F
  VARIANT 8..11: note = may be deleted
  VARIANT 8: note = A, G or V
XXRGXTLXXXX

SEQ ID NO: 288 - protein, 11 aa, synthetic construct
  VARIANT 1: note = G or A
  VARIANT 2: note = Y, F, or W
  VARIANT 9: note = K, N, or Q
  VARIANT 10: note = W or F
  VARIANT 11: note = M, M-NH2, L, I, V, A, or G
  VARIANT 1..2: note = may be deleted
  VARIANT 1: note = may be deleted
  VARIANT 9..11: note = may be deleted
  VARIANT 10..11: note = may be deleted
  VARIANT 11: note = may be deleted
  VARIANT 8..11: note = may be deleted
  VARIANT 8: note = A, G or V
  VARIANT 4: note = G or A
XXRXISLXXXX

SEQ ID NO: 289 - protein, 11 aa, synthetic construct
  VARIANT 1: note = G or A
  VARIANT 2: note = Y, F, or W
  VARIANT 9: note = K, N, or Q
  VARIANT 10: note = W or F
  VARIANT 11: note = M, M-NH2, L, I, V, A, or G
  VARIANT 1..2: note = may be deleted
  VARIANT 1: note = may be deleted
  VARIANT 9..11: note = may be deleted
  VARIANT 10..11: note = may be deleted
  VARIANT 11: note = may be deleted
  VARIANT 8..11: note = may be deleted
  VARIANT 8: note = A, G or V
  VARIANT 4: note = G or A
XXRXITLXXXX

SEQ ID NO: 290 - protein, 11 aa, synthetic construct
  VARIANT 1: note = G or A
  VARIANT 2: note = Y, F, or W
  VARIANT 9: note = K, N, or Q
  VARIANT 10: note = W or F
  VARIANT 11: note = M, M-NH2, L, I, V, A, or G
  VARIANT 1..2: note = may be deleted
  VARIANT 1: note = may be deleted
  VARIANT 9..11: note = may be deleted
  VARIANT 10..11: note = may be deleted
  VARIANT 11: note = may be deleted
  VARIANT 8..11: note = may be deleted
  VARIANT 8: note = A, G or V
  VARIANT 4: note = G or A
XXRXYSLXXXX

SEQ ID NO: 291 - protein, 11 aa, synthetic construct
  VARIANT 1: note = G or A
  VARIANT 2: note = Y, F, or W
  VARIANT 9: note = K, N, or Q
  VARIANT 10: note = W or F
  VARIANT 11: note = M, M-NH2, L, I, V, A, or G
  VARIANT 1..2: note = may be deleted
  VARIANT 1: note = may be deleted
  VARIANT 9..11: note = may be deleted
  VARIANT 10..11: note = may be deleted
  VARIANT 11: note = may be deleted
  VARIANT 8..11: note = may be deleted
  VARIANT 8: note = A, G or V
  VARIANT 4: note = G or A
XXRXYTLXXXX

SEQ ID NO: 292 - protein, 11 aa, synthetic construct
  VARIANT 1: note = G or A
  VARIANT 2: note = Y, F, or W
  VARIANT 9: note = K, N, or Q
  VARIANT 10: note = W or F
  VARIANT 11: note = M, M-NH2, L, I, V, A, or G
  VARIANT 1..2: note = may be deleted
  VARIANT 1: note = may be deleted
  VARIANT 9..11: note = may be deleted
  VARIANT 10..11: note = may be deleted
  VARIANT 11: note = may be deleted
  VARIANT 8..11: note = may be deleted
  VARIANT 8: note = A, G or V
XXRGYSLXXXX

SEQ ID NO: 293 - protein, 11 aa, synthetic construct
  VARIANT 1: note = G or A
  VARIANT 2: note = Y, F, or W
  VARIANT 9: note = K, N, or Q
  VARIANT 10: note = W or F
  VARIANT 11: note = M, M-NH2, L, I, V, A, or G
  VARIANT 1..2: note = may be deleted
  VARIANT 1: note = may be deleted
  VARIANT 9..11: note = may be deleted
  VARIANT 10..11: note = may be deleted
  VARIANT 11: note = may be deleted
  VARIANT 8..11: note = may be deleted
  VARIANT 8: note = A, G or V
XXRGISLXXXX

SEQ ID NO: 294 - protein, 11 aa, synthetic construct
  VARIANT 1: note = G or A
  VARIANT 2: note = Y, F, or W
  VARIANT 9: note = K, N, or Q
  VARIANT 10: note = W or F
  VARIANT 11: note = M, M-NH2, L, I, V, A, or G
  VARIANT 1..2: note = may be deleted
  VARIANT 1: note = may be deleted
  VARIANT 9..11: note = may be deleted
  VARIANT 10..11: note = may be deleted
  VARIANT 11: note = may be deleted
  VARIANT 8..11: note = may be deleted
  VARIANT 8: note = A, G or V
XXRGYTLXXXX

SEQ ID NO: 295 - protein, 11 aa, synthetic construct
  VARIANT 1: note = G or A
  VARIANT 2: note = Y, F, or W
  VARIANT 9: note = K, N, or Q
  VARIANT 10: note = W or F
  VARIANT 11: note = M, M-NH2, L, I, V, A, or G
  VARIANT 1..2: note = may be deleted
  VARIANT 1: note = may be deleted
  VARIANT 9..11: note = may be deleted
  VARIANT 10..11: note = may be deleted
  VARIANT 11: note = may be deleted
  VARIANT 8..11: note = may be deleted
  VARIANT 8: note = A, G or V
XXRGITLXXXX

SEQ ID NO: 296 - protein, 11 aa, synthetic construct
  VARIANT 1: note = G or A
  VARIANT 2: note = Y, F, or W
  VARIANT 9: note = K, N, or Q
  VARIANT 10: note = W or F
  VARIANT 11: note = M, M-NH2, L, I, V, A, or G
  VARIANT 1..2: note = may be deleted
  VARIANT 1: note = may be deleted
  VARIANT 9..11: note = may be deleted
  VARIANT 10..11: note = may be deleted
  VARIANT 11: note = may be deleted
  VARIANT 6: note = S or T
  VARIANT 8..11: note = may be deleted
  VARIANT 8: note = A, G or V
XXKGIXLXXXX

SEQ ID NO: 297 - protein, 11 aa, synthetic construct
  VARIANT 1: note = G or A
  VARIANT 2: note = Y, F, or W
  VARIANT 9: note = K, N, or Q
  VARIANT 10: note = W or F
  VARIANT 11: note = M, M-NH2, L, I, V, A, or G
  VARIANT 1..2: note = may be deleted
  VARIANT 1: note = may be deleted
  VARIANT 9..11: note = may be deleted
  VARIANT 10..11: note = may be deleted
  VARIANT 11: note = may be deleted
  VARIANT 6: note = S or T
  VARIANT 8..11: note = may be deleted
  VARIANT 8: note = A, G or V
XXKGYXLXXXX

SEQ ID NO: 298 - protein, 11 aa, synthetic construct
  VARIANT 1: note = G or A
  VARIANT 2: note = Y, F, or W
  VARIANT 9: note = K, N, or Q
  VARIANT 10: note = W or F
  VARIANT 11: note = M, M-NH2, L, I, V, A, or G
  VARIANT 1..2: note = may be deleted
  VARIANT 1: note = may be deleted
  VARIANT 9..11: note = may be deleted
  VARIANT 10..11: note = may be deleted
  VARIANT 11: note = may be deleted
  VARIANT 5: note = I, Y, Q, N, L, or F
  VARIANT 8..11: note = may be deleted
  VARIANT 8: note = A, G or V
XXKGXSLXXXX

SEQ ID NO: 299 - protein, 11 aa, synthetic construct
  VARIANT 1: note = G or A
  VARIANT 2: note = Y, F, or W
  VARIANT 9: note = K, N, or Q
  VARIANT 10: note = W or F
  VARIANT 11: note = M, M-NH2, L, I, V, A, or G
  VARIANT 1..2: note = may be deleted
  VARIANT 1: note = may be deleted
  VARIANT 9..11: note = may be deleted
  VARIANT 10..11: note = may be deleted
  VARIANT 11: note = may be deleted
  VARIANT 5: note = I, Y, Q, N, L, or F
  VARIANT 8..11: note = may be deleted
  VARIANT 8: note = A, G or V
XXKGXTLXXXX

SEQ ID NO: 300 - protein, 11 aa, synthetic construct
  VARIANT 1: note = G or A
  VARIANT 2: note = Y, F, or W
  VARIANT 9: note = K, N, or Q
  VARIANT 10: note = W or F
  VARIANT 11: note = M, M-NH2, L, I, V, A, or G
  VARIANT 1..2: note = may be deleted
  VARIANT 1: note = may be deleted
  VARIANT 9..11: note = may be deleted
  VARIANT 10..11: note = may be deleted
  VARIANT 11: note = may be deleted
  VARIANT 8..11: note = may be deleted
  VARIANT 8: note = A, G or V
  VARIANT 4: note = G or A
XXKXISLXXXX

SEQ ID NO: 301 - protein, 11 aa, synthetic construct
  VARIANT 1: note = G or A
  VARIANT 2: note = Y, F, or W
  VARIANT 9: note = K, N, or Q
  VARIANT 10: note = W or F
  VARIANT 11: note = M, M-NH2, L, I, V, A, or G
  VARIANT 1..2: note = may be deleted
  VARIANT 1: note = may be deleted
  VARIANT 9..11: note = may be deleted
  VARIANT 10..11: note = may be deleted
  VARIANT 11: note = may be deleted
  VARIANT 8..11: note = may be deleted
  VARIANT 8: note = A, G or V
  VARIANT 4: note = G or A
XXKXITLXXXX

SEQ ID NO: 302 - protein, 11 aa, synthetic construct
  VARIANT 1: note = G or A
  VARIANT 2: note = Y, F, or W
  VARIANT 9: note = K, N, or Q
  VARIANT 10: note = W or F
  VARIANT 11: note = M, M-NH2, L, I, V, A, or G
  VARIANT 1..2: note = may be deleted
  VARIANT 1: note = may be deleted
  VARIANT 9..11: note = may be deleted
  VARIANT 10..11: note = may be deleted
  VARIANT 11: note = may be deleted
  VARIANT 8..11: note = may be deleted
  VARIANT 8: note = A, G or V
  VARIANT 4: note = G or A
XXKXYSLXXXX

SEQ ID NO: 303 - protein, 11 aa, synthetic construct
  VARIANT 1: note = G or A
  VARIANT 2: note = Y, F, or W
  VARIANT 9: note = K, N, or Q
  VARIANT 10: note = W or F
  VARIANT 11: note = M, M-NH2, L, I, V, A, or G
  VARIANT 1..2: note = may be deleted
  VARIANT 1: note = may be deleted
  VARIANT 9..11: note = may be deleted
  VARIANT 10..11: note = may be deleted
  VARIANT 11: note = may be deleted
  VARIANT 8..11: note = may be deleted
  VARIANT 8: note = A, G or V
  VARIANT 4: note = G or A
XXKXYTLXXXX

SEQ ID NO: 304 - protein, 11 aa, synthetic construct
  VARIANT 1: note = G or A
  VARIANT 2: note = Y, F, or W
  VARIANT 9: note = K, N, or Q
  VARIANT 10: note = W or F
  VARIANT 11: note = M, M-NH2, L, I, V, A, or G
  VARIANT 1..2: note = may be deleted
  VARIANT 1: note = may be deleted
  VARIANT 9..11: note = may be deleted
  VARIANT 10..11: note = may be deleted
  VARIANT 11: note = may be deleted
  VARIANT 8..11: note = may be deleted
  VARIANT 8: note = A, G or V
XXKGYSLXXXX

SEQ ID NO: 305 - protein, 11 aa, synthetic construct
  VARIANT 1: note = G or A
  VARIANT 2: note = Y, F, or W
  VARIANT 9: note = K, N, or Q
  VARIANT 10: note = W or F
  VARIANT 11: note = M, M-NH2, L, I, V, A, or G
  VARIANT 1..2: note = may be deleted
  VARIANT 1: note = may be deleted
  VARIANT 9..11: note = may be deleted
  VARIANT 10..11: note = may be deleted
  VARIANT 11: note = may be deleted
  VARIANT 8..11: note = may be deleted
  VARIANT 8: note = A, G or V
XXKGISLXXXX

SEQ ID NO: 306 - protein, 11 aa, synthetic construct
  VARIANT 1: note = G or A
  VARIANT 2: note = Y, F, or W
  VARIANT 9: note = K, N, or Q
  VARIANT 10: note = W or F
  VARIANT 11: note = M, M-NH2, L, I, V, A, or G
  VARIANT 1..2: note = may be deleted
  VARIANT 1: note = may be deleted
  VARIANT 9..11: note = may be deleted
  VARIANT 10..11: note = may be deleted
  VARIANT 11: note = may be deleted
  VARIANT 8..11: note = may be deleted
  VARIANT 8: note = A, G or V
XXKGYTLXXXX

SEQ ID NO: 307 - protein, 11 aa, synthetic construct
  VARIANT 1: note = G or A
  VARIANT 2: note = Y, F, or W
  VARIANT 9: note = K, N, or Q
  VARIANT 10: note = W or F
  VARIANT 11: note = M, M-NH2, L, I, V, A, or G
  VARIANT 1..2: note = may be deleted
  VARIANT 1: note = may be deleted
  VARIANT 9..11: note = may be deleted
  VARIANT 10..11: note = may be deleted
  VARIANT 11: note = may be deleted
  VARIANT 8..11: note = may be deleted
  VARIANT 8: note = A, G or V
XXKGITLXXXX

SEQ ID NO: 308 - protein, 11 aa, synthetic construct
  VARIANT 1: note = G or A
  VARIANT 2: note = Y, F, or W
  VARIANT 9: note = K, N, or Q
  VARIANT 10: note = W or F
  VARIANT 11: note = M, M-NH2, L, I, V, A, or G
  VARIANT 1..2: note = may be deleted
  VARIANT 1: note = may be deleted
  VARIANT 9..11: note = may be deleted
  VARIANT 10..11: note = may be deleted
  VARIANT 11: note = may be deleted
  VARIANT 6: note = S or T
  VARIANT 8..11: note = may be deleted
  VARIANT 8: note = A, G or V
XXLGIXLXXXX

SEQ ID NO: 309 - protein, 11 aa, synthetic construct
  VARIANT 1: note = G or A
  VARIANT 2: note = Y, F, or W
  VARIANT 9: note = K, N, or Q
  VARIANT 10: note = W or F
  VARIANT 11: note = M, M-NH2, L, I, V, A, or G
  VARIANT 1..2: note = may be deleted
  VARIANT 1: note = may be deleted
  VARIANT 9..11: note = may be deleted
  VARIANT 10..11: note = may be deleted
  VARIANT 11: note = may be deleted
  VARIANT 6: note = S or T
  VARIANT 8..11: note = may be deleted
  VARIANT 8: note = A, G or V
XXLGYXLXXXX

SEQ ID NO: 310 - protein, 11 aa, synthetic construct
  VARIANT 1: note = G or A
  VARIANT 8: note = A, G, or V
  VARIANT 9: note = K, N, or Q
  VARIANT 10: note = W or F
  VARIANT 11: note = M, M-NH2, L, I, V, A, or G
  VARIANT 1: note = may be deleted
  VARIANT 8..11: note = may be deleted
  VARIANT 9..11: note = may be deleted
  VARIANT 10..11: note = may be deleted
  VARIANT 11: note = may be deleted
  VARIANT 7..11: note = may be deleted
  VARIANT 7: note = L, I, or V
  VARIANT 6: note = S or T
XFLGIXXXXXX

SEQ ID NO: 311 - protein, 11 aa, synthetic construct
  VARIANT 2: note = Y or F
  VARIANT 3: note = R, K or L
  VARIANT 5: note = I or Y
  VARIANT 6: note = S or T
  VARIANT 9: note = K or N
  VARIANT 11: note = M, M-NH2, or V
  VARIANT 1..3: note = may be deleted
  VARIANT 1..2: note = may be deleted
  VARIANT 1: note = may be deleted
  VARIANT 7..11: note = may be deleted
  VARIANT 8..11: note = may be deleted
  VARIANT 9..11: note = may be deleted
  VARIANT 10..11: note = may be deleted
  VARIANT 11: note = may be deleted
GXXGXXLAXWX

SEQ ID NO: 312 - protein, 11 aa, synthetic construct
GFRGISLANWV

SEQ ID NO: 313 - protein, 11 aa, synthetic construct
  SITE 11: note = Methionine Amide
GFRGISLANWM

SEQ ID NO: 314 - protein, 11 aa, synthetic construct
GYKGISLANWV

SEQ ID NO: 315 - protein, 11 aa, synthetic construct
  SITE 11: note = Methionine Amide
GYKGISLANWM

SEQ ID NO: 316 - protein, 10 aa, synthetic construct
GYRGYSLANW

SEQ ID NO: 317 - protein, 11 aa, synthetic construct
  SITE 11: note = Methionine Amide
GYRGYSLANWM

SEQ ID NO: 318 - protein, 11 aa, synthetic construct
GYRGITLANWV

SEQ ID NO: 319 - protein, 11 aa, synthetic construct
  SITE 11: note = Methionine Amide
GYRGITLANWM

SEQ ID NO: 320 - protein, 11 aa, synthetic construct
GYRGISLAKWV

SEQ ID NO: 321 - protein, 11 aa, synthetic construct
  SITE 11: note = Methionine Amide
GYRGISLAKWM